European Patent Application EP 4 485 466 A2, published January 1, 2025. Title: NOVEL CRISPR ENZYMES AND SYSTEMS. Applicant: The Broad Institute, Inc. Application EP. The sequence listing filed with the application follows.

SEQUENCE LISTING (373 sequences)

SEQ ID NO: 1 - protein, 7 aa, synthetic construct
  REGION 1..7: note = Synthetic
ENLYFQG

SEQ ID NO: 2 - protein, 7 aa, Simian virus 40
PKKKRKV

SEQ ID NO: 3 - protein, 16 aa, synthetic construct
  REGION 1..16: note = Nucleoplasmin bipartite NLS
KRPAATKKAGQAKKKK

SEQ ID NO: 4 - protein, 9 aa, synthetic construct
  REGION 1..9: note = c-myc NLS from Homo sapiens
PAAKRVKLD

SEQ ID NO: 5 - protein, 11 aa, synthetic construct
  REGION 1..11: note = c-myc NLS from Homo sapiens
RQRRNELKRSP

SEQ ID NO: 6 - protein, 38 aa, synthetic construct
  REGION 1..38: note = hRNPA1 M9 NLS from Homo sapiens
NQSSNFGPMKGGNFGGRSSGPYGGGGQYFAKPRNQGGY

SEQ ID NO: 7 - protein, 42 aa, synthetic construct
  REGION 1..42: note = IBB domain from importin-alpha from Homo sapiens
RMRIZFKNKGKDTAELRRRRVEVSVELRKAKKDEQILKRRNV

SEQ ID NO: 8 - protein, 8 aa, synthetic construct
  REGION 1..8: note = Myoma T protein from Homo sapiens
VSRKRPRP

SEQ ID NO: 9 - protein, 8 aa, synthetic construct
  REGION 1..8: note = Myoma T protein from Homo sapiens
PPKKARED

SEQ ID NO: 10 - protein, 8 aa, Homo sapiens
PQPKKKPL

SEQ ID NO: 11 - protein, 12 aa, Mus sp.
SALIKKKKKMAP

SEQ ID NO: 12 - protein, 5 aa, Influenza virus
DRLRR

SEQ ID NO: 13 - protein, 7 aa, Influenza virus
PKQKKRK

SEQ ID NO: 14 - protein, 10 aa, Hepatitis D virus
RKLKKKIKKL

SEQ ID NO: 15 - protein, 10 aa, Mus sp.
REKKKFLKRR

SEQ ID NO: 16 - protein, 20 aa, Homo sapiens
KRKGDEVDGVDEVAKKKSKK

SEQ ID NO: 17 - protein, 17 aa, Homo sapiens
RKCLQAGMNLEARKTKK

SEQ ID NO: 18 - protein, 4 aa, synthetic construct
  REGION 1..4: note = GlySer Linker
GGGS

SEQ ID NO: 19 - protein, 15 aa, synthetic construct
  REGION 1..15: note = GlySer Linker
GGGGSGGGGSGGGGS

SEQ ID NO: 20 - protein, 30 aa, synthetic construct
  REGION 1..30: note = GlySer Linker
GGGGSGGGGSGGGGSGGGGSGGGGSGGGGS

SEQ ID NO: 21 - protein, 45 aa, synthetic construct
  REGION 1..45: note = GlySer Linker
GGGGSGGGGSGGGGSGGGGSGGGGSGGGGSGGGGSGGGGSGGGGS

SEQ ID NO: 22 - protein, 60 aa, synthetic construct
  REGION 1..60: note = GlySer Linker
GGGGSGGGGSGGGGSGGGGSGGGGSGGGGSGGGGSGGGGSGGGGSGGGGSGGGGSGGGGS

SEQ ID NO: 23 - DNA, 20 bp, synthetic construct
  misc_feature 1..20: note = Synthetic Oligonucleotide
  source 1..20: mol_type = other DNA
gagtccgagcagaagaagaa

SEQ ID NO: 24 - DNA, 20 bp, synthetic construct
  misc_feature 1..20: note = Synthetic Oligonucleotide
  source 1..20: mol_type = other DNA
gagtcctagcaggagaagaa

SEQ ID NO: 25 - DNA, 20 bp, synthetic construct
  misc_feature 1..20: note = Synthetic Oligonucleotide
  source 1..20: mol_type = other DNA
gagtctaagcagaagaagaa

SEQ ID NO: 26 - protein, 9 aa, synthetic construct
  REGION 1..9: note = Synthetic Peptide
LAGLIDADG

SEQ ID NO: 27 - DNA, 32 bp, synthetic construct
  misc_feature 1..32: note = Synthetic Oligonucleotide
  source 1..32: mol_type = other DNA
ggtaagacgtctcggtcgtctccgtccgtttc

SEQ ID NO: 28 - DNA, 32 bp, synthetic construct
  misc_feature 1..32: note = Synthetic Oligonucleotide
  source 1..32: mol_type = other DNA
agacgctctgttgggactctgggcggcatttt

SEQ ID NO: 29 - DNA, 32 bp, synthetic construct
  misc_feature 1..32: note = Synthetic Oligonucleotide
  source 1..32: mol_type = other DNA
ttttctgtccctgcttatcctgtccactctct

SEQ ID NO: 30 - DNA, 23 bp, Homo sapiens
  source 1..23: mol_type = other DNA
tacatacccaccaccgtgcctgg

SEQ ID NO: 31 - DNA, 23 bp, Homo sapiens
  source 1..23: mol_type = other DNA
tagacgcccaccaccatgcctgg

SEQ ID NO: 32 - DNA, 23 bp, Homo sapiens
  source 1..23: mol_type = other DNA
tagatgcccaccaccgtgcctgg

SEQ ID NO: 33 - DNA, 23 bp, Homo sapiens
  source 1..23: mol_type = other DNA
tagacgcccaccaccgtgcctgg

SEQ ID NO: 34 - DNA, 23 bp, Homo sapiens
  source 1..23: mol_type = other DNA
tagacacccaccaccatgcctgg

SEQ ID NO: 35 - DNA, 24 bp, Homo sapiens
  source 1..24: mol_type = other DNA
ctgatggtccatggtctgttactc

SEQ ID NO: 36 - DNA, 23 bp, Homo sapiens
  source 1..23: mol_type = other DNA
ctgatggtccatggtctgttact

SEQ ID NO: 37 - DNA, 14 bp, Homo sapiens
  source 1..14: mol_type = other DNA
ctgatggtccatgg

SEQ ID NO: 38 - protein, 1325 aa, Acidaminococcus sp. BV3L6
MTQFEGFTNLYQVSKTLRFELIPQGKTLKHIQEQGFIEEDKARNDHYKELKPIIDRIYKTYADQCLQLVQLDWENLSAAIDSYRKEKTEETRNALIEEQATYRNAIHDYFIGRTDNLTDAINKRHAEIYKGLFKAELFNGKVLKQLGTVTTTEHENALLRSFDKFTTYFSGFYENRKNVFSAEDISTAIPHRIVQDNFPKFKENCHIFTRLITAVPSLREHFENVKKAIGIFVSTSIEEVFSFPFYNQLLTQTQIDLYNQLLGGISREAGTEKIKGLNEVLNLAIQKNDETAHIIASLPHRFIPLFKQILSDRNTLSFILEEFKSDEEVIQSFCKYKTLLRNENVLETAEALFNELNSIDLTHIFISHKKLETISSALCDHWDTLRNALYERRISELTGKITKSAKEKVQRSLKHEDINLQEIISAAGKELSEAFKQKTSEILSHAHAALDQPLPTTLKKQEEKEILKSQLDSLLGLYHLLDWFAVDESNEVDPEFSARLTGIKLEMEPSLSFYNKARNYATKKPYSVEKFKLNFQMPTLASGWDVNKEKNNGAILFVKNGLYYLGIMPKQKGRYKALSFEPTEKTSEGFDKMYYDYFPDAAKMIPKCSTQLKAVTAHFQTHTTPILLSNNFIEPLEITKEIYDLNNPEKEPKKFQTAYAKKTGDQKGYREALCKWIDFTRDFLSKYTKTTSIDLSSLRPSSQYKDLGEYYAELNPLLYHISFQRIAEKEIMDAVETGKLYLFQIYNKDFAKGHHGKPNLHTLYWTGLFSPENLAKTSIKLNGQAELFYRPKSRMKRMAHRLGEKMLNKKLKDQKTPIPDTLYQELYDYVNHRLSHDLSDEARALLPNVITKEVSHEIIKDRRFTSDKFFFHVPITLNYQAANSPSKFNQRVNAYLKEHPETPIIGIDRGERNLIYITVIDSTGKILEQRSLNTIQQFDYQKKLDNREKERVAARQAWSVVGTIKDLKQGYLSQVIHEIVDLMIHYQAVVVLENLNFGFKSKRTGIAEKAVYQQFEKMLIDKLNCLVLKDYPAEKVGGVLNPYQKYDAVIALEDLNSGFKNSRVKVLTDQFTSFAKMGTQSGFLFYVPAPYTSKIDPLTGFVDPFVWKTIKNHESRKHFLEGFDFLHYDVKTGDFILHFKMNRNLSFQRGLPGFMPAWDIVFEKNETQFDAKGTPFIAGKRIVPVIENHRFTGRYRDLYPANELIALLEEKGIVFRDGSNILPKLLENDDSHAIDTMVALIRSVLQMRNSNAATGEDYINSPVRDLNGVCFDSRFQNPEWPMDADANGAYHIALKGQLLLNHLKESKDLKLQNGISNQDWLAYIQ

SEQ ID NO: 39 - protein, 1201 aa, Lachnospiraceae bacterium ND2006
MSKLEKFTNCYSLSKTLRFKAIPVGKTQENIDNKRLLVEDEKRAEDYKGVKKLLDRYYLSFINDVLHSIKLKNLNNYISLFRKKTRTEKENKELENLEINLRKEIAKAFKGNEGYKSLFKKDIIETILPEFLDDKDEIALVNSFNGFTTAFTGFFDNRENMFSEEAKSTSIAFRCINENLTRYISNMDIFEKVDAIFDKHEVQEIKEKILNSDYDVEDFFEGEFFNFVLTQEGIDVYNAIIGGFVTESGEKIKGLNEYINLYNQKTKQKLPKFKPLYKQVLSDRESLSFYGEGYTSDEEVLEVFRNTLNKNSEIFSSIKKLEKLFKNFDEYSSAGIFVKNGPAISTISKDIFGEWNVIRDKWNAEYDDIHLKKKAVVTEKYEDDRRKSFKKIGSFSLEQLQEYADADLSVVEKLKEIIIQKVDEIYKVYGSSEKLFDADFVLEKSLKKNDAVVAIMKDLLDSVKSFENYIKAFFGEGKETNRDESFYGDFVLAYDILLKVDHIYDAIRNYVTQKPYSKDKFKLYFQNPQFMGGWDKDKETDYRATILRYGSKYYLAIMDKKYAKCLQKIDKDDVNGNYEKINYKLLPGPNKMLPKVFFSKKWMAYYNPSEDIQKIYKNGTFKKGDMFNLNDCHKLIDFFKDSISRYPKWSNAYDFNFSETEKYKDIAGFYREVEEQGYKVSFESASKKEVDKLVEEGKLYMFQIYNKDFSDKSHGTPNLHTMYFKLLFDENNHGQIRLSGGAELFMRRASLKKEELVVHPANSPIANKNPDNPKKTTTLSYDVYKDKRFSEDQYELHIPIAINKCPKNIFKINTEVRVLLKHDDNPYVIGIDRGERNLLYIVVVDGKGNIVEQYSLNEIINNFNGIRIKTDYHSLLDKKEKERFEARQNWTSIENIKELKAGYISQVVHKICELVEEKQVYQKFEKMLIDKLNYMVDKKSNPCATGGALKGYQITNKFESFKSMSTQNGFIFYIPAWLTSKIDPSTGFVNLLKTKYTSIADSKKFISSFDRIMYVPEEDLFEFALDYKNFSRTDADYIKKWKLYSYGNRIRIFRNPKKNNVFDWEEVCLTSAYKELFNKYGINYQQGDIRALLCEQSDKAFYSSFMALMSLMLQMRNSITGRTDVDFLISPVKNSDGIFYDSRNYEAQENAILPKNADANGAYNIARKVLWAIGQFKKAEDEKLDKVKIAISNKEWLEYAQ

SEQ ID NO: 40 - DNA, 27 bp, synthetic construct
  misc_feature 1..27: note = Synthetic Oligonucleotide
  source 1..27: mol_type = other DNA
tttgctaggaatattgaagggggcagg

SEQ ID NO: 41 - DNA, 27 bp, synthetic construct
  misc_feature 1..27: note = Synthetic Oligonucleotide
  source 1..27: mol_type = other DNA
caagccaggaatattaaaaggggttgg

SEQ ID NO: 42 - DNA, 27 bp, synthetic construct
  misc_feature 1..27: note = Synthetic Oligonucleotide
  source 1..27: mol_type = other DNA
aaggctaggaagctgggaggtggcagg

SEQ ID NO: 43 - DNA, 27 bp, synthetic construct
  misc_feature 1..27: note = Synthetic Oligonucleotide
  source 1..27: mol_type = other DNA
catagcaggtattttgaagggggcagg

SEQ ID NO: 44 - DNA, 27 bp, synthetic construct
  misc_feature 1..27: note = Synthetic Oligonucleotide
  source 1..27: mol_type = other DNA
tttggtgctcaatgaaaggagataagg

SEQ ID NO: 45 - DNA, 27 bp, synthetic construct
  misc_feature 1..27: note = Synthetic Oligonucleotide
  source 1..27: mol_type = other DNA
tttgaagaaatattacaacatataaaa

SEQ ID NO: 46 - DNA, 26 bp, synthetic construct
  misc_feature 1..26: note = Synthetic Oligonucleotide
  source 1..26: mol_type = other DNA
tccaaataaattttacacatttaaaa

SEQ ID NO: 47 - DNA, 28 bp, synthetic construct
  misc_feature 1..28: note = Synthetic Oligonucleotide
  source 1..28: mol_type = other DNA
gagaaagaaacattacctaatgataaaa

SEQ ID NO: 48 - DNA, 28 bp, synthetic construct
  misc_feature 1..28: note = Synthetic Oligonucleotide
  source 1..28: mol_type = other DNA
aacaaagaaatattagaaaataattaaa

SEQ ID NO: 49 - DNA, 28 bp, synthetic construct
  misc_feature 1..28: note = Synthetic Oligonucleotide
  source 1..28: mol_type = other DNA
cataaacaaatatcactaatatataaaa

SEQ ID NO: 50 - DNA, 27 bp, synthetic construct
  misc_feature 1..27: note = Synthetic Oligonucleotide
  source 1..27: mol_type = other DNA
gagaaaaaaatattaatacatatacag

SEQ ID NO: 51 - DNA, 27 bp, synthetic construct
  misc_feature 1..27: note = Synthetic Oligonucleotide
  source 1..27: mol_type = other DNA
tttgtcctccggttctggaaccacacc

SEQ ID NO: 52 - DNA, 27 bp, synthetic construct
  misc_feature 1..27: note = Synthetic Oligonucleotide
  source 1..27: mol_type = other DNA
ttcatcctccggttctggaaccagatt

SEQ ID NO: 53 - DNA, 27 bp, synthetic construct
  misc_feature 1..27: note = Synthetic Oligonucleotide
  source 1..27: mol_type = other DNA
ttcatcctccggttctggaaccagatc

SEQ ID NO: 54 - DNA, 27 bp, synthetic construct
  misc_feature 1..27: note = Synthetic Oligonucleotide
  source 1..27: mol_type = other DNA
ttcatcctccggttctgaaaccacact

SEQ ID NO: 55 - DNA, 27 bp, synthetic construct
  misc_feature 1..27: note = Synthetic Oligonucleotide
  source 1..27: mol_type = other DNA
ttcatcctccggttctgaaaccagatc

SEQ ID NO: 56 - DNA, 27 bp, synthetic construct
  misc_feature 1..27: note = Synthetic Oligonucleotide
  source 1..27: mol_type = other DNA
ttcatcctctggttctggaaccaggtc

SEQ ID NO: 57 - DNA, 27 bp, synthetic construct
  misc_feature 1..27: note = Synthetic Oligonucleotide
  source 1..27: mol_type = other DNA
ttcatccttcggttctggaaccagatc

SEQ ID NO: 58 - DNA, 27 bp, synthetic construct
  misc_feature 1..27: note = Synthetic Oligonucleotide
  source 1..27: mol_type = other DNA
cctctcctctggttctggaacactgaa

SEQ ID NO: 59 - DNA, 27 bp, synthetic construct
  misc_feature 1..27: note = Synthetic Oligonucleotide
  source 1..27: mol_type = other DNA
tttggggtgatcagacccaacagcagg

SEQ ID NO: 60 - DNA, 27 bp, synthetic construct
  misc_feature 1..27: note = Synthetic Oligonucleotide
  source 1..27: mol_type = other DNA
tttggggtgatcagacccaacaccagg

SEQ ID NO: 61 - DNA, 27 bp, synthetic construct
  misc_feature 1..27: note = Synthetic Oligonucleotide
  source 1..27: mol_type = other DNA
tttggggtgatcagacccaaccccagg

SEQ ID NO: 62 - DNA, 27 bp, synthetic construct
  misc_feature 1..27: note = Synthetic Oligonucleotide
  source 1..27: mol_type = other DNA
tttggggtgatcaggcccaacaccagg

SEQ ID NO: 63 - DNA, 27 bp, synthetic construct
  misc_feature 1..27: note = Synthetic Oligonucleotide
  source 1..27: mol_type = other DNA
tttgtcctccggttctggaaccacacc

SEQ ID NO: 64 - DNA, 27 bp, synthetic construct
  misc_feature 1..27: note = Synthetic Oligonucleotide
  source 1..27: mol_type = other DNA
ttcatcctccggttctggaaccagatt

SEQ ID NO: 65 - DNA, 27 bp, synthetic construct
  misc_feature 1..27: note = Synthetic Oligonucleotide
  source 1..27: mol_type = other DNA
ttcatcctccggttctggaaccagatc

SEQ ID NO: 66 - DNA, 27 bp, synthetic construct
  misc_feature 1..27: note = Synthetic Oligonucleotide
  source 1..27: mol_type = other DNA
ttcatcctccggttctgaaaccacact

SEQ ID NO: 67 - DNA, 27 bp, synthetic construct
  misc_feature 1..27: note = Synthetic Oligonucleotide
  source 1..27: mol_type = other DNA
ttcatcctccggttctgaaaccagatc

SEQ ID NO: 68 - DNA, 27 bp, synthetic construct
  misc_feature 1..27: note = Synthetic Oligonucleotide
  source 1..27: mol_type = other DNA
ttcatcctctggttctggaaccaggtc

SEQ ID NO: 69 - DNA, 27 bp, synthetic construct
  misc_feature 1..27: note = Synthetic Oligonucleotide
  source 1..27: mol_type = other DNA
ttcatccttcggttctggaaccagatc

SEQ ID NO: 70 - protein, 5 aa, synthetic construct
  REGION 1..5: note = GlySer Linker
GGGGS

SEQ ID NO: 71 - protein, 10 aa, synthetic construct
  REGION 1..10: note = GlySer Linker
GGGGSGGGGS

SEQ ID NO: 72 - protein, 12 aa, synthetic construct
  REGION 1..12: note = Synthetic Peptide
FWYHKMILVAGC

SEQ ID NO: 73 - protein, 12 aa, synthetic construct
  REGION 1..12: note = Synthetic Peptide
WYHKREDCSTNQ

SEQ ID NO: 74 - protein, 9 aa, synthetic construct
  REGION 1..9: note = Synthetic Peptide
VCAGSPTND

SEQ ID NO: 75 - protein, 4 aa, synthetic construct
  REGION 1..4: note = Synthetic Peptide
FWYH

SEQ ID NO: 76 - skipped

SEQ ID NO: 77 - protein, 5 aa, synthetic construct
  REGION 1..5: note = Synthetic Peptide
HKRED

SEQ ID NO: 78-81 - skipped (4 entries)

SEQ ID NO: 82 - protein, 20 aa, synthetic construct
  REGION 1..20: note = GlySer Linker
GGGGSGGGGSGGGGSGGGGS

SEQ ID NO: 83 - protein, 25 aa, synthetic construct
  REGION 1..25: note = GlySer Linker
GGGGSGGGGSGGGGSGGGGSGGGGS

SEQ ID NO: 84 - skipped

SEQ ID NO: 85 - protein, 35 aa, synthetic construct
  REGION 1..35: note = GlySer Linker
GGGGSGGGGSGGGGSGGGGSGGGGSGGGGSGGGGS

SEQ ID NO: 86 - protein, 40 aa, synthetic construct
  REGION 1..40: note = GlySer Linker
GGGGSGGGGSGGGGSGGGGSGGGGSGGGGSGGGGSGGGGS

SEQ ID NO: 87 - protein, 50 aa, synthetic construct
  REGION 1..50: note = GlySer Linker
GGGGSGGGGSGGGGSGGGGSGGGGSGGGGSGGGGSGGGGSGGGGSGGGGS

SEQ ID NO: 88 - protein, 55 aa, synthetic construct
  REGION 1..55: note = GlySer Linker
GGGGSGGGGSGGGGSGGGGSGGGGSGGGGSGGGGSGGGGSGGGGSGGGGSGGGGS

SEQ ID NO: 89 - DNA, 20 bp, Homo sapiens
  source 1..20: mol_type = other DNA
gccaaattggacgaccctcg

SEQ ID NO: 90 - DNA, 20 bp, Homo sapiens
  source 1..20: mol_type = other DNA
cgaggagacccccgtttcgg

SEQ ID NO: 91 - DNA, 20 bp, Homo sapiens
  source 1..20: mol_type = other DNA
cccgccgccgccgtggctcg

SEQ ID NO: 92 - DNA, 20 bp, Homo sapiens
  source 1..20: mol_type = other DNA
tgagctctacgagatccaca

SEQ ID NO: 93 - DNA, 20 bp, synthetic construct
  misc_feature 1..20: note = Synthetic Oligonucleotide
  source 1..20: mol_type = other DNA
ggtctcatgtgtggcactca

SEQ ID NO: 94 - DNA, 20 bp, synthetic construct
  misc_feature 1..20: note = Synthetic Oligonucleotide
  source 1..20: mol_type = other DNA
tgtccaaccttcaggcaagg

SEQ ID NO: 95 - DNA, 21 bp, synthetic construct
  misc_feature 1..21: note = Synthetic Oligonucleotide
  source 1..21: mol_type = other DNA
gtaacgtcctggacactgtgg

SEQ ID NO: 96 - DNA, 21 bp, synthetic construct
  misc_feature 1..21: note = Synthetic Oligonucleotide
  source 1..21: mol_type = other DNA
ttggtccaataggtcatgacg

SEQ ID NO: 97 - DNA, 22 bp, synthetic construct
  misc_feature 1..22: note = Synthetic Oligonucleotide
  source 1..22: mol_type = other DNA
tggctaagcctggccaagaacg

SEQ ID NO: 98 - DNA, 22 bp, synthetic construct
  misc_feature 1..22: note = Synthetic Oligonucleotide
  source 1..22: mol_type = other DNA
tcaggatgaaggctgccttcgg

SEQ ID NO: 99 - DNA, 485 bp, Homo sapiens
  source 1..485: mol_type = other DNA
gtgtctagactgcagagggccctgcgtatgagtgcaagtgggttttaggaccaggatgaggcggggtgggggtgcctacctgacgaccgaccccgacccactggacaagcacccaacccccattccccaaattgcgcatcccctatcagagagggggaggggaaacaggatgcggcgaggcgcgtgcgcactgccagcttcagcaccgcggacagtgccttcgcccccgcctggcggcgcgcgccaccgccgcctcagcactgaaggcgcgctgacgtcactcgccggtcccccgcaaactccccttcccggccaccttggtcgcgtccgcgccgccgccggcccagccggaccgcaccacgcgaggcgcgagataggggggcacgggcgcgaccatctgcgctgcggcgccggcgactcagcgctgcctcagtctgcggtgggcagcggaggagtcgtgtcgtgcctgagagcgcagtcgagaa

SEQ ID NO: 100 - DNA, 229 bp, Mus sp.
  source 1..229: mol_type = other DNA
agctgaatggggtccgcctcttttccctgcctaaacagacaggaactcctgccaattgagggcgtcaccgctaaggctccgccccagcctgggctccacaaccaatgaagggtaatctcgacaaagagcaaggggtggggcgcgggcgcgcaggtgcagcagcacacaggctggtcgggagggcggggcgcgacgtctgccgtgcggggtcccggcatcggttgcgcgc

SEQ ID NO: 101 - DNA, 30 bp, unidentified
  misc_feature 1..30: note = Synthetic Oligonucleotide
  source 1..30: mol_type = other DNA
atgtacccatacgatgttccagattacgct

SEQ ID NO: 102 - DNA, 33 bp, unidentified
  misc_feature 1..33: note = Synthetic Oligonucleotide
  source 1..33: mol_type = other DNA
tcgccgaagaaaaagcgcaaggtcgaagcgtcc

SEQ ID NO: 103 - DNA, 48 bp, unidentified
  misc_feature 1..48: note = Synthetic Oligonucleotide
  source 1..48: mol_type = other DNA
aataaaagatctttattttcattagatctgtgtgttggttttttgtgt

SEQ ID NO: 104 - DNA, 72 bp, unidentified
  misc_feature 1..72: note = Synthetic Oligonucleotide
  source 1..72: mol_type = other DNA
ggctcgttggtctaggggtatgattctcgcttagggtgcgagaggtcccgggttcaaatcccggacgagccc

SEQ ID NO: 105 - DNA, 249 bp, unidentified
  misc_feature 1..249: note = Synthetic Oligonucleotide
  source 1..249: mol_type = other DNA
gagggcctatttcccatgattccttcatatttgcatatacgatacaaggctgttagagagataattggaattaatttgactgtaaacacaaagatattagtacaaaatacgtgacgtagaaagtaataatttcttgggtagtttgcagttttaaaattatgttttaaaatggactatcatatgcttaccgtaacttgaaagtatttcgatttcttggctttatatatcttgtggaaaggacgaaacacc

SEQ ID NO: 106 - DNA, 49 bp, unidentified
  misc_feature 1..49: note = Synthetic Oligonucleotide
  source 1..49: mol_type = other DNA
gtaatttctactgttgtagatggaagagcatatatgctcttcttttttt

SEQ ID NO: 107 - DNA, 122 bp, synthetic construct
  misc_feature 1..122: note = Synthetic Oligonucleotide
  source 1..122: mol_type = other DNA
aacacaggaccggtgccaccatgtacccatacgatgttccagattacgcttcgccgaagaaaaagcgcaaggtcgaagcgtccacacagttcgagggctttaccaacctgtatcaggtgagc

SEQ ID NO: 108 - DNA, 94 bp, unidentified
  misc_feature 1..94: note = Synthetic Oligonucleotide
  source 1..94: mol_type = other DNA
gcggccgcacacaaaaaaccaacacacagatctaatgaaaataaagatcttttattgaattcttagttgcgcagctcctggatgtaggccagcc

SEQ ID NO: 109 - DNA, 118 bp, unidentified
  misc_feature 1..118: note = Synthetic Oligonucleotide
  source 1..118: mol_type = other DNA
taccggatccccgggtaccggtatgtacccatacgatgttccagattacgcttcgccgaagaaaaagcgcaaggtcgaagcgtccagcaagctggagaagtttacaaactgctactcc

SEQ ID NO: 110 - DNA, 115 bp, unidentified
  misc_feature 1..115: note = Synthetic Oligonucleotide
  source 1..115: mol_type = other DNA
gcggccgcacacaaaaaaccaacacacagatctaatgaaaataaagatcttttattgaattcttagtgcttcacgctggtctgggcgtactccagccactccttgttagagatgg

SEQ ID NO: 111 - DNA, 397 bp, Mus musculus
  source 1..397: mol_type = other DNA
cctacgctagcctgagggcctatttcccatgattccttcatatttgcatatacgatacaaggctgttagagagataattggaattaatttgactgtaaacacaaagatattagtacaaaatacgtgacgtagaaagtaataatttcttgggtagtttgcagttttaaaattatgttttaaaatggactatcatatgcttaccgtaacttgaaagtatttcgatttcttggctttatatatcttgtggaaaggacgaaacaccgtaatttctactcttgtagatcctgcctctgctggctctgctaatttctactcttgtagatcggcgggtctcagggttgtctaatttctactcttgtagattgtccctgcttatcctgtccttttttcgacgcgt

SEQ ID NO: 112 - DNA, 397 bp, Mus sp.
  source 1..397: mol_type = other DNA
cctacgctagcctgagggcctatttcccatgattccttcatatttgcatatacgatacaaggctgttagagagataattggaattaatttgactgtaaacacaaagatattagtacaaaatacgtgacgtagaaagtaataatttcttgggtagtttgcagttttaaaattatgttttaaaatggactatcatatgcttaccgtaacttgaaagtatttcgatttcttggctttatatatcttgtggaaaggacgaaacaccgtaatttctactcttgtagatttcgccttcttaaacttcagtaatttctactcttgtagatgtgtccctatggtaggtccctaatttctactcttgtagattcatctctttagctgtgtcattttttcgacgcgt

SEQ ID NO: 113 - DNA, 316 bp, unidentified
  misc_feature 1..316: note = Synthetic Oligonucleotide
  source 1..316: mol_type = other DNA
ccctacgctagcctgagggcctatttcccatgattccttcatatttgcatatacgatacaaggctgttagagagataattggaattaatttgactgtaaacacaaagatattagtacaaaatacgtgacgtagaaagtaataatttcttgggtagtttgcagttttaaaattatgttttaaaatggactatcatatgcttaccgtaacttgaaagtatttcgatttcttggctttatatatcttgtggaaaggacgaaacaccgtaatttctactcttgtagatgaagagcgagctcttcttttttcgacgcgtgt

SEQ ID NO: 114 - DNA, 23 bp, synthetic construct
  misc_feature 1..23: note = Synthetic Oligonucleotide
  source 1..23: mol_type = other DNA
ctgatggtccatgtctgttactc

SEQ ID NO: 115 - DNA, 23 bp, synthetic construct
  misc_feature 1..23: note = Synthetic Oligonucleotide
  source 1..23: mol_type = other DNA
tggttgcccaccctagtcattgg

SEQ ID NO: 116 - DNA, 23 bp, synthetic construct
  misc_feature 1..23: note = Synthetic Oligonucleotide
  source 1..23: mol_type = other DNA
ctaggaatattgaagggggcagg

SEQ ID NO: 117 - DNA, 23 bp, synthetic construct
  misc_feature 1..23: note = Synthetic Oligonucleotide
  source 1..23: mol_type = other DNA
gtgctcaatgaaaggagataagg

SEQ ID NO: 118 - DNA, 57 bp, synthetic construct
  misc_feature 1..57: note = Synthetic Oligonucleotide
  source 1..57: mol_type = other DNA
agatctgatggtccatgtctgttactcaatttctactcttgtagattggttgcccac

SEQ ID NO: 119 - DNA, 96 bp, synthetic construct
  misc_feature 1..96: note = Synthetic Oligonucleotide
  source 1..96: mol_type = other DNA
cctagtcattggaatttctactcttgtagatctaggaatattgaagggggcaggaatttctactcttgtagatgtgctcaatgaaaggagataagg

SEQ ID NO: 120 - DNA, 57 bp, synthetic construct
  misc_feature 1..57: note = Synthetic Oligonucleotide
  source 1..57: mol_type = other DNA
aaaaccttatctcctttcattgagcacatctacaagagtagaaattcctgccccctt

SEQ ID NO: 121 - DNA, 96 bp, synthetic construct
  misc_feature 1..96: note = Synthetic Oligonucleotide
  source 1..96: mol_type = other DNA
caatattcctagatctacaagagtagaaattccaatgactagggtgggcaaccaatctacaagagtagaaattgagtaacagacatggaccatcag

SEQ ID NO: 122 - DNA, 71 bp, synthetic construct
  misc_feature 1..71: note = Synthetic Oligonucleotide
  source 1..71: mol_type = other DNA
agatctgatggtccatgtctgttactcgcctgtcaatttctactcttgtagattggttgcccaccctagtc

SEQ ID NO: 123 - DNA, 42 bp, synthetic construct
  misc_feature 1..42: note = Synthetic Oligonucleotide
  source 1..42: mol_type = other DNA
acactggcccggggctgggacgtgaataaggagaagaacaat

SEQ ID NO: 124 - DNA, 42 bp, synthetic construct
  misc_feature 1..42: note = Synthetic
  source 1..42: mol_type = other DNA
acactggcctcaggctgggacgtgaagaaggagaagaacaat

SEQ ID NO: 125 - DNA, 42 bp, synthetic construct; identical to SEQ ID NO: 124
  misc_feature 1..42: note = Synthetic Oligonucleotide
  source 1..42: mol_type = other DNA

SEQ ID NO: 126 - DNA, 42 bp, synthetic construct
  misc_feature 1..42: note = Synthetic Oligonucleotide
  source 1..42: mol_type = other DNA
acactggcctcaggctgggacgtgaatgccgagaagaacaat

SEQ ID NO: 127 - DNA, 42 bp, synthetic construct
  misc_feature 1..42: note = Synthetic Oligonucleotide
  source 1..42: mol_type = other DNA
acactggcctcaggctgggacgtgaatcacgagaagaacaat

SEQ ID NO: 128 - DNA, 42 bp, synthetic construct
  misc_feature 1..42: note = Synthetic Oligonucleotide
  source 1..42: mol_type = other DNA
acactggcctcaggctgggacgtgaataacgagaagaacaat

SEQ ID NO: 129 - DNA, 42 bp, synthetic construct
  misc_feature 1..42: note = Synthetic Oligonucleotide
  source 1..42: mol_type = other DNA
acactggcctcaggctgggacgtgaatcaggagaagaacaat

SEQ ID NO: 130 - skipped

SEQ ID NO: 131 - DNA, 42 bp, synthetic construct
  misc_feature 1..42: note = Synthetic Oligonucleotide
  source 1..42: mol_type = other DNA
acactggcctcaggctgggacgtgaataaggagtacaacaat

SEQ ID NO: 132 - DNA, 42 bp, synthetic construct
  misc_feature 1..42: note = Synthetic Oligonucleotide
  source 1..42: mol_type = other DNA
acactggcctcaggctgggacgtgaataaggagaagcggaat

SEQ ID NO: 133 - DNA, 42 bp, synthetic construct
  misc_feature 1..42: note = Synthetic Oligonucleotide
  source 1..42: mol_type = other DNA
acactggcctcaggctgggacgtgaataaggagaagaacggc

SEQ ID NO: 134 - DNA, 42 bp, synthetic construct
  misc_feature 1..42: note = Synthetic Oligonucleotide
  source 1..42: mol_type = other DNA
acactggcctcaggctgggacgtgaataaggagaagaacaag

SEQ ID NO: 135 - DNA, 42 bp, synthetic construct
  misc_feature 1..42: note = Synthetic Oligonucleotide
  source 1..42: mol_type = other DNA
acactggcctcaggctgggacgtgaataaggagaagaaccgg

SEQ ID NO: 136 - DNA, 42 bp, synthetic construct
  misc_feature 1..42: note = Synthetic Oligonucleotide
  source 1..42: mol_type = other DNA
acactggcctcaggctgggacgtgaataaggagaagaacagc

SEQ ID NO: 137 - DNA, 42 bp, synthetic construct
  misc_feature 1..42: note = Synthetic Oligonucleotide
  source 1..42: mol_type = other DNA
acactggcctcaggctgggacgtgaataaggagaagaacacc

SEQ ID NO: 138 - DNA, 44 bp, synthetic construct
  misc_feature 1..44: note = Synthetic Oligonucleotide
  source 1..44: mol_type = other DNA
atgccgccaagatgatcccagcctgcagcacccagctgaaggcg

SEQ ID NO: 139 - DNA, 44 bp, synthetic construct
  misc_feature 1..44: note = Synthetic Oligonucleotide
  source 1..44: mol_type = other DNA
atgccgccaagatgatcccacggtgcagcacccagctgaaggcg

SEQ ID NO: 140 - DNA, 42 bp, synthetic construct
  misc_feature 1..42: note = Synthetic Oligonucleotide
  source 1..42: mol_type = other DNA
acactggcccggggctgggacgtgaatcgggagaagaacaat

SEQ ID NO: 141 - DNA, 42 bp, synthetic construct
  misc_feature 1..42: note = Synthetic Oligonucleotide
  source 1..42: mol_type = other DNA
acactggcctcaggctgggacgtgaatcgggagaagaaccgg

SEQ ID NO: 142 - DNA, 42 bp, synthetic construct
  misc_feature 1..42: note = Synthetic Oligonucleotide
  source 1..42: mol_type = other DNA
acactggcccggggctgggacgtgaataaggagtacaacaat

SEQ ID NO: 143 - DNA, 42 bp, synthetic construct
  misc_feature 1..42: note = Synthetic Oligonucleotide
  source 1..42: mol_type = other DNA
acactggcccggggctgggacgtgaatcgggagtacaacaat

SEQ ID NO: 144 - DNA, 42 bp, synthetic construct
  misc_feature 1..42: note = Synthetic Oligonucleotide
  source 1..42: mol_type = other DNA
cggctggcctcaggctgggacgtgaataaggagaagaacaat

SEQ ID NO: 145 - DNA, 42 bp, synthetic construct
  misc_feature 1..42: note = Synthetic Oligonucleotide
  source 1..42: mol_type = other DNA
aagctggcctcaggctgggacgtgaataaggagaagaacaat

SEQ ID NO: 146 - DNA, 42 bp, synthetic construct
  misc_feature 1..42: note = Synthetic Oligonucleotide
  source 1..42: mol_type = other DNA
acactggcctcaggctgggacgtgaatggcgagaagaacaat

SEQ ID NO: 147 - DNA, 42 bp, synthetic construct
  misc_feature 1..42: note = Synthetic Oligonucleotide
  source 1..42: mol_type = other DNA
acactggcctcaggctgggacgtgaattgcgagaagaacaat

SEQ ID NO: 148 - DNA, 42 bp, synthetic construct
  misc_feature 1..42: note = Synthetic Oligonucleotide
  source 1..42: mol_type = other DNA
acactggcctcaggctgggacgtgaatttcgagaagaacaat

SEQ ID NO: 149 - DNA, 42 bp, synthetic construct
  misc_feature 1..42: note = Synthetic Oligonucleotide
  source 1..42: mol_type = other DNA
acactggcctcaggctgggacgtgaatatcgagaagaacaat

SEQ ID NO: 150 - DNA, 42 bp, synthetic construct
  misc_feature 1..42: note = Synthetic Oligonucleotide
  source 1..42: mol_type = other DNA
acactggcctcaggctgggacgtgaatatggagaagaacaat

SEQ ID NO: 151 - DNA, 42 bp, synthetic construct
  misc_feature 1..42: note = Synthetic Oligonucleotide
  source 1..42: mol_type = other DNA
acactggcctcaggctgggacgtgaatagcgagaagaacaat

SEQ ID NO: 152 - DNA, 42 bp, synthetic construct
  misc_feature 1..42: note = Synthetic Oligonucleotide
  source 1..42: mol_type = other DNA
acactggcctcaggctgggacgtgaataccgagaagaacaat

SEQ ID NO: 153 - DNA, 42 bp, synthetic construct
  misc_feature 1..42: note = Synthetic Oligonucleotide
  source 1..42: mol_type = other DNA
acactggcctcaggctgggacgtgaatgtggagaagaacaat

SEQ ID NO: 154 - DNA, 42 bp, synthetic construct
  misc_feature 1..42: note = Synthetic Oligonucleotide
  source 1..42: mol_type = other DNA
acactggcctcaggctgggacgtgaattgggagaagaacaat

SEQ ID NO: 155 - DNA, 42 bp, synthetic construct
  misc_feature 1..42: note = Synthetic Oligonucleotide
  source 1..42: mol_type = other DNA
acactggcctcaggctgggacgtgaattacgagaagaacaat

SEQ ID NO: 156 - DNA, 42 bp, synthetic construct
  misc_feature 1..42: note = Synthetic Oligonucleotide
  source 1..42: mol_type = other DNA
acactggcctcaggctgggacgtgaatgacgagaagaacaat

SEQ ID NO: 157 - DNA, 42 bp, synthetic construct
  misc_feature 1..42: note = Synthetic Oligonucleotide
  source 1..42: mol_type = other DNA
acactggcctcaggctgggacgtgaatgaggagaagaacaat

SEQ ID NO: 158 - DNA, 42 bp, synthetic construct
  misc_feature 1..42: note = Synthetic Oligonucleotide
  source 1..42: mol_type = other DNA
acactggcctcaggctgggacgtgaatctggagaagaacaat

SEQ ID NO: 159 - DNA, 42 bp, synthetic construct
  misc_feature 1..42: note = Synthetic Oligonucleotide
  source 1..42: mol_type = other DNA
acactggcctcaggctgggacgtgaatcccgagaagaacaat

SEQ ID NO: 160 - DNA, 42 bp, synthetic construct
  misc_feature 1..42: note = Synthetic Oligonucleotide
  source 1..42: mol_type = other DNA
acactggcccggggctgggacgtgaatgtggagaagaacaat

SEQ ID NO: 161 - DNA, 42 bp, synthetic construct
  misc_feature 1..42: note = Synthetic Oligonucleotide
  source 1..42: mol_type = other DNA
acactggcctcaggctgggacgtgaatgtggagaagaaccgg

SEQ ID NO: 162 - DNA, 42 bp, synthetic construct
  misc_feature 1..42: note = Synthetic Oligonucleotide
  source 1..42: mol_type = other DNA
acactggcccggggctgggacgtgaatgtggagaagaaccgg

SEQ ID NO: 163 - DNA, 42 bp, synthetic construct
  misc_feature 1..42: note = Synthetic Oligonucleotide
  source 1..42: mol_type = other DNA
acactggcccggggctgggacgtgaatgtggagaagcggcgg

SEQ ID NO: 164 - DNA, 42 bp, synthetic construct
  misc_feature 1..42: note = Synthetic Oligonucleotide
  source 1..42: mol_type = other DNA
acactggcccggggctgggacgtgaagaaggagaagaacaat

SEQ ID NO: 165 - DNA, 42 bp, synthetic construct; identical to SEQ ID NO: 160
  misc_feature 1..42: note = Synthetic Oligonucleotide
  source 1..42: mol_type = other DNA

SEQ ID NO: 166 - DNA, 42 bp, synthetic construct
  misc_feature 1..42: note = Synthetic Oligonucleotide
  source 1..42: mol_type = other DNA
acactggcccggggctgggacgtgaataaggagaagcggaat

SEQ ID NO: 167 - DNA, 42 bp, synthetic construct
  misc_feature 1..42: note = Synthetic Oligonucleotide
  source 1..42: mol_type = other DNA
acactggcccggggctgggacgtgaataaggagaagaacagc

SEQ ID NO: 168 - DNA, 42 bp, synthetic construct
  misc_feature 1..42: note = Synthetic
  source 1..42: mol_type = other DNA
acactggcccggggctgggacgtgaagaaggagtacaacaat

SEQ ID NO: 169 - DNA, 42 bp, synthetic construct
  misc_feature 1..42: note = Synthetic Oligonucleotide
  source 1..42: mol_type = other DNA
acactggcccggggctgggacgtgaagaaggagaagcggaat

SEQ ID NO: 170 - DNA, 42 bp, synthetic construct
  misc_feature 1..42: note = Synthetic Oligonucleotide
  source 1..42: mol_type = other DNA
acactggcccggggctgggacgtgaagaaggagaagaacagc

SEQ ID NO: 171 - DNA, 42 bp, synthetic construct
  misc_feature 1..42: note = Synthetic Oligonucleotide
  source 1..42: mol_type = other DNA
acactggcccggggctgggacgtgaataaggagtaccggaat

SEQ ID NO: 172 - DNA, 42 bp, synthetic construct
  misc_feature 1..42: note = Synthetic Oligonucleotide
  source 1..42: mol_type = other DNA
acactggcccggggctgggacgtgaataaggagtacaacagc

SEQ ID NO: 173 - DNA, 42 bp, synthetic construct
  misc_feature 1..42: note = Synthetic Oligonucleotide
  source 1..42: mol_type = other DNA
acactggcccggggctgggacgtgaataaggagaagcggagc

SEQ ID NO: 174 - DNA, 42 bp, synthetic construct
  misc_feature 1..42: note = Synthetic Oligonucleotide
  source 1..42: mol_type = other DNA
acactggcccggggctgggacgtgaagaaggagtaccggagc

SEQ ID NO: 175 - DNA, 42 bp, synthetic construct
  misc_feature 1..42: note = Synthetic Oligonucleotide
  source 1..42: mol_type = other DNA
acactggcctcaggctgggacgtgaatgtggagaagaacggc

SEQ ID NO: 176 - DNA, 42 bp, synthetic construct
  misc_feature 1..42: note = Synthetic Oligonucleotide
  source 1..42: mol_type = other DNA
acactggcccggggctgggacgtgaatgtggagaagaacggc

SEQ ID NO: 177 - DNA, 42 bp, synthetic construct
  misc_feature 1..42: note = Synthetic Oligonucleotide
  source 1..42: mol_type = other DNA
acactggcccggggctgggacgtgaatgtggagaagcggggc

SEQ ID NO: 178 - DNA, 23 bp, Acidaminococcus sp. BV3L6
  source 1..23: mol_type = other DNA
aaggaggaggaagctgctaagga

SEQ ID NO: 179 - DNA, 23 bp, Acidaminococcus sp. BV3L6
  source 1..23: mol_type = other DNA
actagggtgggcaaccacaaacc

SEQ ID NO: 180 - DNA, 23 bp, Acidaminococcus sp. BV3L6
  source 1..23: mol_type = other DNA
cctctttagccagagccggggtg

SEQ ID NO: 181 - DNA, 23 bp, Acidaminococcus sp. BV3L6
  source 1..23: mol_type = other DNA
agggcgttggagcggggagaagg

SEQ ID NO: 182 - DNA, 23 bp, Acidaminococcus sp. BV3L6
  source 1..23: mol_type = other DNA
gagcggggagaaggccaggggtc

SEQ ID NO: 183 - DNA, 23 bp, Acidaminococcus sp. BV3L6
  source 1..23: mol_type = other DNA
aaattccagcaccgagcgccctg

SEQ ID NO: 184 - DNA, 23 bp, Acidaminococcus sp. BV3L6
  source 1..23: mol_type = other DNA
tagctgtttgggaggtcagaaat

SEQ ID NO: 185 - DNA, 23 bp, Acidaminococcus sp. BV3L6
  source 1..23: mol_type = other DNA
tctttagccagagccggggtgtg

SEQ ID NO: 186 - DNA, 23 bp, Acidaminococcus sp. BV3L6
  source 1..23: mol_type = other DNA
cgctccaacgccctcaaccccac

SEQ ID NO: 187 - DNA, 23 bp, Acidaminococcus sp. BV3L6
  source 1..23: mol_type = other DNA
tggccaggctttggggaggcctg

SEQ ID NO: 188 - DNA, 23 bp, Acidaminococcus sp. BV3L6
  source 1..23: mol_type = other DNA
tctgtcaatggcggccccgggct

SEQ ID NO: 189 - DNA, 23 bp, Acidaminococcus sp. BV3L6
  source 1..23: mol_type = other DNA
gtcacccctgtttctggcaccag

SEQ ID NO: 190 - DNA, 23 bp, Acidaminococcus sp. BV3L6
  source 1..23: mol_type = other DNA
cccgctccaacgccctcaacccc

SEQ ID NO: 191 - DNA, 23 bp, Acidaminococcus sp. BV3L6
  source 1..23: mol_type = other DNA
gctaaagagggaatgggctttgg

SEQ ID NO: 192 - DNA, 23 bp, Acidaminococcus sp. BV3L6
  source 1..23: mol_type = other DNA
tgtgggtgagtgagtgtgtgcgt

SEQ ID NO: 193 - DNA, 23 bp, Acidaminococcus sp. BV3L6
  source 1..23: mol_type = other DNA
ccctcccgtcacccctgtttctg

SEQ ID NO: 194 - DNA, 23 bp, Acidaminococcus sp. BV3L6
  source 1..23: mol_type = other DNA
aatggcggccccgggcttcaagc

SEQ ID NO: 195 - DNA, 23 bp, Acidaminococcus sp. BV3L6
  source 1..23: mol_type = other DNA
ggtgagtgagtgtgtgcgtgtgg

SEQ ID NO: 196 - DNA, 23 bp, Acidaminococcus sp. BV3L6
  source 1..23: mol_type = other DNA
aaagcccattccctctttagcca

SEQ ID NO: 197 - DNA, 23 bp, Acidaminococcus sp. BV3L6
  source 1..23: mol_type = other DNA
ctctttagccagagccggggtgt

SEQ ID NO: 198 - DNA, 23 bp, Acidaminococcus sp. BV3L6
  source 1..23: mol_type = other DNA
tggtgccagaaacaggggtgacg

SEQ ID NO: 199 - DNA, 23 bp, Acidaminococcus sp. BV3L6
  source 1..23: mol_type = other DNA
ctgatggtccatgtctgttactc

SEQ ID NO: 200 - DNA, 23 bp, Acidaminococcus sp. BV3L6
  source 1..23: mol_type = other DNA
gctgaagggaaataaaaggaaaa

SEQ ID NO: 201 - DNA, 23 bp, Acidaminococcus sp. BV3L6
  source 1..23: mol_type = other DNA
gccaccacagggaagctgggtga

SEQ ID NO: 202 - DNA, 23 bp, Acidaminococcus sp. BV3L6
  source 1..23: mol_type = other DNA
aattccagcaccgagcgccctgg

SEQ ID NO: 203 - DNA, 23 bp, Acidaminococcus sp. BV3L6
  source 1..23: mol_type = other DNA
aaaattttacaccacaaaatgtt

SEQ ID NO: 204 - DNA, 23 bp, Acidaminococcus sp. BV3L6
  source 1..23: mol_type = other DNA
tatttctgacctcccaaacagct

SEQ ID NO: 205 - DNA, 23 bp, Acidaminococcus sp. BV3L6
  source 1..23: mol_type = other DNA
atgaatatcaaattccagcaccg

SEQ ID NO: 206 - DNA, 23 bp, Acidaminococcus sp. BV3L6
  source 1..23: mol_type = other DNA
catcaaccggtggcgcattgcca

SEQ ID NO: 207 - DNA, 23 bp, Acidaminococcus sp. BV3L6
  source 1..23: mol_type = other DNA
gagccggggtgtgcagacggcag

SEQ ID NO: 208 - DNA, 23 bp, Acidaminococcus sp. BV3L6
  source 1..23: mol_type = other DNA
ttaaagaaaatatcatctttggt

SEQ ID NO: 209 - DNA, 23 bp, Acidaminococcus sp. BV3L6
  source 1..23: mol_type = other DNA
agcgccccctagtgactgccgtc

SEQ ID NO: 210 - DNA, 23 bp, Acidaminococcus sp. BV3L6
  source 1..23: mol_type = other DNA
tccccattggcctgcttcgtggc

SEQ ID NO: 211 - DNA, 23 bp, Acidaminococcus sp. BV3L6
  source 1..23: mol_type = other DNA
gtcagcggactcaccggccaggg

SEQ ID NO: 212 - DNA, 23 bp, Acidaminococcus sp. BV3L6
  source 1..23: mol_type = other DNA
ttccctctttagccagagccggg

SEQ ID NO: 213 - DNA, 23 bp, Acidaminococcus sp. BV3L6
  source 1..23: mol_type = other DNA
ggcttcaagccctgtggggccat

SEQ ID NO: 214 - DNA, 23 bp, Acidaminococcus sp. BV3L6
  source 1..23: mol_type = other DNA
aagatgatattttctttaatggt

SEQ ID NO: 215 - DNA, 23 bp, Acidaminococcus sp. BV3L6
  source 1..23: mol_type = other DNA
ctgtggtggccgagcgcccccta

SEQ ID NO: 216 - DNA, 23 bp, Acidaminococcus sp. BV3L6
  source 1..23: mol_type = other DNA
tctgcacaccccggctctggcta

SEQ ID NO: 217 - DNA, 23 bp, Acidaminococcus sp. BV3L6
  source 1..23: mol_type = other DNA
atgtcctccccattggcctgctt

SEQ ID NO: 218 - DNA, 23 bp, Acidaminococcus sp. BV3L6
  source 1..23: mol_type = other DNA
caaatatgtagctgtttgggagg

SEQ ID NO: 219 - DNA, 23 bp, Acidaminococcus sp. BV3L6
  source 1..23: mol_type = other DNA
ctccattcacccagcttccctgt

SEQ ID NO: 220 - DNA, 23 bp, Acidaminococcus sp. BV3L6
  source 1..23: mol_type = other DNA
aggaaaactgagaacagaatgaa

SEQ ID NO: 221 - DNA, 23 bp, Acidaminococcus sp. BV3L6
  source 1..23: mol_type = other DNA
taaactcattaatgcccttcggc

SEQ ID NO: 222 - DNA, 23 bp, Acidaminococcus sp. BV3L6
  source 1..23: mol_type = other DNA
atgtcacctccaatgactagggt

SEQ ID NO: 223 - DNA, 23 bp, Acidaminococcus sp. BV3L6
  source 1..23: mol_type = other DNA
tggcaatgcgccaccggttgatg

SEQ ID NO: 224 - DNA, 23 bp, Acidaminococcus sp. BV3L6
  source 1..23: mol_type = other DNA
gcgatgttttttctggagattta

SEQ ID NO: 225 - DNA, 23 bp, Acidaminococcus sp. BV3L6
  source 1..23: mol_type = other DNA
cagggaagctgggtgaatggagc

SEQ ID NO: 226 - DNA, 23 bp, Acidaminococcus sp. BV3L6
  source 1..23: mol_type = other DNA
ccacagggaagctgggtgaatgg

SEQ ID NO: 227 - DNA, 23 bp, Acidaminococcus sp. BV3L6
  source 1..23: mol_type = other DNA
gggtgtgcagacggcagtcacta

SEQ ID NO: 228 - DNA, 23 bp, Acidaminococcus sp. BV3L6
  source 1..23: mol_type = other DNA
tgggctctctgtacatgaagcaa

SEQ ID NO: 229 - DNA, 23 bp, Acidaminococcus sp. BV3L6
  source 1..23: mol_type = other DNA
gaaatagggggtccaggagcaaa

SEQ ID NO: 230 - DNA, 23 bp, Acidaminococcus sp. BV3L6
  source 1..23: mol_type = other DNA
cctagtgactgccgtctgcacac

SEQ ID NO: 231 - DNA, 23 bp, Acidaminococcus sp. BV3L6
  source 1..23: mol_type = other DNA
gccagggcgctcggtgctggaat

SEQ ID NO: 232 - DNA, 23 bp, Acidaminococcus sp. BV3L6
  source 1..23: mol_type = other DNA
attccctctttagccagagccgg

SEQ ID NO: 233 - DNA, 23 bp, Acidaminococcus sp. BV3L6
  source 1..23: mol_type = other DNA
gctctggctaaagagggaatggg

SEQ ID NO: 234 - DNA, 23 bp, Acidaminococcus sp. BV3L6
  source 1..23: mol_type = other DNA
cggctctggctaaagagggaatg

SEQ ID NO: 235 - DNA, 23 bp, Acidaminococcus sp. BV3L6
  source 1..23: mol_type = other DNA
tcactctcgaagacgctgctcgc

SEQ ID NO: 236 - DNA, 23 bp, Acidaminococcus sp. BV3L6
  source 1..23: mol_type = other DNA
gcttccctgtggtggccgagcgc

SEQ ID NO: 237 - DNA, 23 bp, Acidaminococcus sp. BV3L6
  source 1..23: mol_type = other DNA
agtcccaaatatgtagctgtttg

SEQ ID NO: 238 - DNA, 23 bp, Acidaminococcus sp. BV3L6
  source 1..23: mol_type = other DNA
ccccctttccaaagcccattccc

SEQ ID NO: 239 - DNA, 23 bp, Acidaminococcus sp. BV3L6
  source 1..23: mol_type = other DNA
aagacgctgctcgctccattcac

SEQ ID NO: 240 - DNA, 23 bp, Acidaminococcus sp. BV3L6
  source 1..23: mol_type = other DNA
gtccacctaaccgctgcgcctcc

SEQ ID NO: 241 - DNA, 23 bp, Acidaminococcus sp. BV3L6
  source 1..23: mol_type = other DNA
tggaccccctatttctgacctcc

SEQ ID NO: 242 - DNA, 23 bp, Acidaminococcus sp. BV3L6
  source 1..23: mol_type = other DNA
ggaggcgcagcggttaggtggac

SEQ ID NO: 243 - DNA, 23 bp, Acidaminococcus sp. BV3L6
  source 1..23: mol_type = other DNA
cctatttctgacctcccaaacag

SEQ ID NO: 244 - DNA, 23 bp, Acidaminococcus sp. BV3L6
  source 1..23: mol_type = other DNA
tctttagccagagccggggtgtg

SEQ ID NO: 245 - DNA, 23 bp, Acidaminococcus sp. BV3L6
  source 1..23: mol_type = other DNA
gtcccaaatatgtagctgtttgg

SEQ ID NO: 246 - DNA, 23 bp, Acidaminococcus sp. BV3L6
  source 1..23: mol_type = other DNA
ctagggggcgctcggccaccaca

SEQ ID NO: 247 - DNA, 23 bp, Acidaminococcus sp. BV3L6
  source 1..23: mol_type = other DNA
cctttccaaagcccattccctct

SEQ ID NO: 248 - DNA, 23 bp, Acidaminococcus sp. BV3L6
  source 1..23: mol_type = other DNA
ctccaacgccctcaaccccacac

SEQ ID NO: 249 - DNA, 23 bp, Acidaminococcus sp. BV3L6
  source 1..23: mol_type = other DNA
ctctttagccagagccggggtgt

SEQ ID NO: 250 - DNA, 23 bp, Acidaminococcus sp. BV3L6
  source 1..23: mol_type = other DNA
cacgtaacctcactttcctgctc

SEQ ID NO: 251 - DNA, 23 bp, Acidaminococcus sp. BV3L6
  source 1..23: mol_type = other DNA
ccccaccccctttccaaagccca

SEQ ID NO: 252 - DNA, 23 bp, Acidaminococcus sp. BV3L6
  source 1..23: mol_type = other DNA
gtcacccctgtttctggcaccag

SEQ ID NO: 253 - DNA, 23 bp, Acidaminococcus sp. BV3L6
  source 1..23: mol_type = other DNA
tggtgccagaaacaggggtgacg

SEQ ID NO: 254 - DNA, 23 bp, Acidaminococcus sp. BV3L6
  source 1..23: mol_type = other DNA
gctaaaataaaggaggaggaagc

SEQ ID NO: 255 - DNA, 23 bp, Acidaminococcus sp. BV3L6
  source 1..23: mol_type = other DNA
cccccggaaactctgtccagaga

SEQ ID NO: 256 - DNA, 23 bp, Acidaminococcus sp. BV3L6
  source 1..23: mol_type = other DNA
atagatctgtgtgtccctctccc

SEQ ID NO: 257 - DNA, 23 bp, Acidaminococcus sp. BV3L6
  source 1..23: mol_type = other DNA
gtctccgtgaacgttcccttagc

SEQ ID NO: 258 - DNA, 23 bp, Acidaminococcus sp. BV3L6
  source 1..23: mol_type = other DNA
tggagtgacccctggccttctcc

SEQ ID NO: 259 - DNA, 23 bp, Acidaminococcus sp. BV3L6
  source 1..23: mol_type = other DNA
aaagcccattccctctttagcca

SEQ ID NO: 260 - DNA, 23 bp, Acidaminococcus sp. BV3L6
  source 1..23: mol_type = other DNA
ctttccaaagcccattccctctt

SEQ ID NO: 261 - DNA, 23 bp, Acidaminococcus sp. BV3L6
  source 1..23: mol_type = other DNA
ggggcggatgggtaattttcagg

SEQ ID NO: 262 - DNA, 23 bp, Acidaminococcus sp. BV3L6
  source 1..23: mol_type = other DNA
cggagactgaacactcctcaaac

SEQ ID NO: 263 - DNA, 23 bp, Acidaminococcus sp. BV3L6
  source 1..23: mol_type = other DNA
cccaccccctttccaaagcccat

SEQ ID NO: 264 - DNA, 23 bp, Acidaminococcus sp. BV3L6
  source 1..23: mol_type = other DNA
ccaccccctttccaaagcccatt

SEQ ID NO: 265 - DNA, 30 bp, Homo sapiens
  source 1..30: mol_type = other DNA
ccgatggtccatgtctgttactcgcctgtc

SEQ ID NO: 266 - DNA, 23 bp, Homo sapiens
  source 1..23: mol_type = other DNA
aaattccagcaccgagcgccctg

SEQ ID NO: 267 - DNA, 23 bp, Homo sapiens
  source 1..23: mol_type = other DNA
aagaaatattacaacatataaaa

SEQ ID NO: 268 - DNA, 23 bp, Homo sapiens
  source 1..23: mol_type = other DNA
gtcacccctgtttctggcaccag

SEQ ID NO: 269 - DNA, 23 bp, Homo sapiens
  source 1..23: mol_type = other DNA
tggtgccagaaacaggggtgacg

SEQ ID NO: 270 - DNA, 24 bp, Homo sapiens
  source 1..24: mol_type = other DNA
gagaagtcatttaataaggccact

SEQ ID NO: 271 - DNA, 23 bp, Homo sapiens
  source 1..23: mol_type = other DNA
gcagttgtcgcagttttacaacc

SEQ ID NO: 272 - DNA, 23 bp, Homo sapiens
  source 1..23: mol_type = other DNA
acccggataacaaggaggaacgc

SEQ ID NO: 273 - DNA, 23 bp, Homo sapiens
  source 1..23: mol_type = other DNA
gagttgattggattgagaataga

SEQ ID NO: 274 - DNA, 23 bp, Homo sapiens
  source 1..23: mol_type = other DNA
gcctctccctgctcagaatctgg

SEQ ID NO: 275 - DNA, 23 bp, Homo sapiens
  source 1..23: mol_type = other DNA
tagctgtttgggaggtcagaaat

SEQ ID NO: 276 - DNA, 23 bp, Homo sapiens
  source 1..23: mol_type = other DNA
gacatgtcccatttgtgggaact

SEQ ID NO: 277 - DNA, 23 bp, Homo sapiens
  source 1..23: mol_type = other DNA
ttcgggtgctgtgaacttccctc

SEQ ID NO: 278 - DNA, 23 bp, Homo sapiens
  source 1..23: mol_type = other DNA
acccactgcgtgggttcccatga

SEQ ID NO: 279 - DNA, 23 bp, Homo sapiens
  source 1..23: mol_type = other DNA
ccaagtcaaacttctcttcagtc

SEQ ID NO: 280 - DNA, 23 bp, Homo sapiens
  source 1..23: mol_type = other DNA
ccctttaggacacatgctgtcta

SEQ ID NO: 281 - DNA, 23 bp, Homo sapiens
  source 1..23: mol_type = other DNA
agtgcaccttcggcgtgctgcag

SEQ ID NO: 282 - DNA, 23 bp, Homo sapiens
  source 1..23: mol_type = other DNA
cccaccatgacaggaagaacggc

SEQ ID NO: 283 - DNA, 23 bp, Homo sapiens
  source 1..23: mol_type = other DNA
aggcgcttccccagcacaaactg

SEQ ID NO: 284 - DNA, 23 bp, Homo sapiens
  source 1..23: mol_type = other DNA
gcgatgttttttctggagattta

SEQ ID NO: 285 - DNA, 23 bp, Homo sapiens
  source 1..23: mol_type = other DNA
gctaaaataaaggaggaggaagc

SEQ ID NO: 286 - DNA, 23 bp, Homo sapiens
  source 1..23: mol_type = other DNA
gtcacccctgtttctggcaccag

SEQ ID NO: 287 - DNA, 23 bp, Homo sapiens
  source 1..23: mol_type = other DNA
tggtgccagaaacaggggtgacg

SEQ ID NO: 288 - DNA, 23 bp, Homo sapiens
  source 1..23: mol_type = other DNA
gtctccgtgaacgttcccttagc

SEQ ID NO: 289 - DNA, 23 bp, Homo sapiens
  source 1..23: mol_type = other DNA
cggagactgaacactcctcaaac

SEQ ID NO: 290 - DNA, 23 bp, Homo sapiens
  source 1..23: mol_type = other DNA
tggcaatgcgccaccggttgatg

SEQ ID NO: 291 - DNA, 23 bp, Homo sapiens
  source 1..23: mol_type = other DNA
ctgtggtggccgagcgcccccta

SEQ ID NO: 292 - DNA, 23 bp, Homo sapiens
  source 1..23: mol_type = other DNA
gtcccaaatatgtagctgtttgg

SEQ ID NO: 293 - DNA, 23 bp, Homo sapiens
  source 1..23: mol_type = other DNA
cacgtaacctcactttcctgctc

SEQ ID NO: 294 - DNA, 23 bp, Homo sapiens
  source 1..23: mol_type = other DNA
tctttagccagagccggggtgtg

SEQ ID NO: 295 - DNA, 23 bp, Homo sapiens
  source 1..23: mol_type = other DNA
cccccggaaactctgtccagaga

SEQ ID NO: 296 - DNA, 23 bp, Homo sapiens
  source 1..23: mol_type = other DNA
ggggcggatgggtaattttcagg

SEQ ID NO: 297 - DNA, 23 bp, Homo sapiens
  source 1..23: mol_type = other DNA
atagatctgtgtgtccctctccc

SEQ ID NO: 298 - DNA, 23 bp, Homo sapiens
  source 1..23: mol_type = other DNA
aaagcccattccctctttagcca

SEQ ID NO: 299 - DNA, 23 bp, Homo sapiens
  source 1..23: mol_type = other DNA
cccaccccctttccaaagcccat

SEQ ID NO: 300 - DNA, 23 bp, Homo sapiens
  source 1..23: mol_type = other DNA
aaaattttacaccacaaaatgtt

SEQ ID NO: 301 - DNA, 23 bp, Homo sapiens
  source 1..23: mol_type = other DNA
aagatgatattttctttaatggt

SEQ ID NO: 302 - DNA, 23 bp, Homo sapiens
  source 1..23: mol_type = other DNA
ttaaagaaaatatcatctttggt

SEQ ID NO: 303 - DNA, 23 bp, Homo sapiens
  source 1..23: mol_type = other DNA
taaactcattaatgcccttcggc

SEQ ID NO: 304 - DNA, 23 bp, Homo sapiens
  source 1..23: mol_type = other DNA
aggaaaactgagaacagaatgaa

SEQ ID NO: 305 - DNA, 23 bp, Homo sapiens
  source 1..23: mol_type = other DNA
catcaaccggtggcgcattgcca

SEQ ID NO: 306 - DNA, 23 bp, Homo sapiens
  source 1..23: mol_type = other DNA
tccccattggcctgcttcgtggc

SEQ ID NO: 307 - DNA, 23 bp, Homo sapiens
  source 1..23: mol_type = other DNA
ggcttcaagccctgtggggccat

SEQ ID NO: 308 - DNA, 23 bp, Homo sapiens
  source 1..23: mol_type = other DNA
atgtcacctccaatgactagggt

SEQ ID NO: 309 - DNA, 23 bp, Homo sapiens
  source 1..23: mol_type = other DNA
atgtcctccccattggcctgctt

SEQ ID NO: 310 - DNA, 23 bp, Homo sapiens
  source 1..23: mol_type = other DNA
ttccctctttagccagagccggg

SEQ ID NO: 311 - DNA, 23 bp, Homo sapiens
  source 1..23: mol_type = other DNA
gccaccacagggaagctgggtga

SEQ ID NO: 312 - DNA, 23 bp, Homo sapiens
  source 1..23: mol_type = other DNA
caaatatgtagctgtttgggagg

SEQ ID NO: 313 - DNA, 23 bp, Homo sapiens
  source 1..23: mol_type = other DNA
agcgccccctagtgactgccgtc

SEQ ID NO: 314 - DNA, 23 bp, Homo sapiens
  source 1..23: mol_type = other DNA
attccctctttagccagagccgg

SEQ ID NO: 315 - DNA, 23 bp, Homo sapiens
  source 1..23: mol_type = other DNA
gctctggctaaagagggaatggg

SEQ ID NO: 316 - DNA, 23 bp, Homo sapiens
  source 1..23: mol_type = other DNA
gagccggggtgtgcagacggcag

SEQ ID NO: 317 - DNA, 23 bp, Homo sapiens
  source 1..23: mol_type = other DNA
ctccattcacccagcttccctgt

SEQ ID NO: 318 - DNA, 23 bp, Homo sapiens
  source 1..23: mol_type = other DNA
gaaatagggggtccaggagcaaa

SEQ ID NO: 319 - DNA, 23 bp, Homo sapiens
  source 1..23: mol_type = other DNA
agtcccaaatatgtagctgtttg

SEQ ID NO: 320 - DNA, 23 bp, Homo sapiens
  source 1..23: mol_type = other DNA
tgggctctctgtacatgaagcaa

SEQ ID NO: 321 - DNA, 23 bp, Homo sapiens
  source 1..23: mol_type = other DNA
cagggaagctgggtgaatggagc

SEQ ID NO: 322 - DNA, 23 bp, Homo sapiens
  source 1..23: mol_type = other DNA
cggctctggctaaagagggaatg

SEQ ID NO: 323 - DNA, 23 bp, Homo sapiens
  source 1..23: mol_type = other DNA
gcttccctgtggtggccgagcgc

SEQ ID NO: 324 - DNA, 23 bp, Homo sapiens
  source 1..23: mol_type = other DNA
tctgcacaccccggctctggcta

SEQ ID NO: 325 - DNA, 23 bp, Homo sapiens
  source 1..23: mol_type = other DNA
cctagtgactgccgtctgcacac

SEQ ID NO: 326 - DNA, 23 bp, Homo sapiens
  source 1..23: mol_type = other DNA
cctatttctgacctcccaaacag

SEQ ID NO: 327 - DNA, 23 bp, Homo sapiens
  source 1..23: mol_type = other DNA
ccacagggaagctgggtgaatgg

SEQ ID NO: 328 - DNA, 23 bp, Homo sapiens
  source 1..23: mol_type = other DNA
tcactctcgaagacgctgctcgc

SEQ ID NO: 329 - DNA, 23 bp, Homo sapiens
  source 1..23: mol_type = other DNA
ctagggggcgctcggccaccaca

SEQ ID NO: 330 - DNA, 23 bp, Homo sapiens
  source 1..23: mol_type = other DNA
gggtgtgcagacggcagtcacta

SEQ ID NO: 331 - DNA, 23 bp, Homo sapiens
  source 1..23: mol_type = other DNA
aagacgctgctcgctccattcac

SEQ ID NO: 332 - DNA, 23 bp, Homo sapiens
  source 1..23: mol_type = other DNA
ctccaacgccctcaaccccacac

SEQ ID NO: 333 - DNA, 23 bp, Homo sapiens
  source 1..23: mol_type = other DNA
tggaccccctatttctgacctcc

SEQ ID NO: 334 - DNA, 23 bp, Homo sapiens
  source 1..23: mol_type = other DNA
tggagtgacccctggccttctcc

SEQ ID NO: 335 - DNA, 23 bp, Homo sapiens
  source 1..23: mol_type = other DNA
cctttccaaagcccattccctct

SEQ ID NO: 336 - DNA, 23 bp, Homo sapiens
  source 1..23: mol_type = other DNA
ccaccccctttccaaagcccatt

SEQ ID NO: 337 - DNA, 23 bp, Homo sapiens
  source 1..23: mol_type = other DNA
ctaggaatattgaagggggcagg

SEQ ID NO: 338 - DNA, 23 bp, Homo sapiens
  source 1..23: mol_type = other DNA
gtgctcaatgaaaggagataagg

SEQ ID NO: 339 - DNA, 23 bp, Homo sapiens
  source 1..23: mol_type = other DNA
aagaaatattacaacatataaaa

SEQ ID NO: 340 - DNA, 23 bp, Homo sapiens
  source 1..23: mol_type = other DNA
tcctccggttctggaaccacacc

SEQ ID NO: 341 - DNA, 23 bp, Homo sapiens
  source 1..23: mol_type = other DNA
gggtgatcagacccaacagcagg

SEQ ID NO: 342 - DNA, 23 bp, Homo sapiens
  source 1..23: mol_type = other DNA
atggtgccaggcataatccagga

SEQ ID NO: 343 - DNA, 23 bp, Homo sapiens
  source 1..23: mol_type = other DNA
ccttcagctaaaataaaggagga

SEQ ID NO: 344 - DNA, 23 bp, Homo sapiens
  source 1..23: mol_type = other DNA
aggagtgttcagtctccgtgaac

SEQ ID NO: 345 - DNA, 23 bp, Homo sapiens
  source 1..23: mol_type = other DNA
ctgatggtccatgtctgttactc

SEQ ID NO: 346 - DNA, 23 bp, Homo sapiens
  source 1..23: mol_type = other DNA
gctgaagggaaataaaaggaaaa

SEQ ID NO: 347 - DNA, 23 bp, Homo sapiens
  source 1..23: mol_type = other DNA
gggaggcctggagtcatggcccc

SEQ ID NO: 348 - DNA, 23 bp, Homo sapiens
  source 1..23: mol_type = other DNA
tggttgcccaccctagtcattgg

SEQ ID NO: 349 - DNA, 23 bp, Homo sapiens
  source 1..23: mol_type = other DNA
gccagagccggggtgtgcagacg

SEQ ID NO: 350 - DNA, 23 bp, Homo sapiens
  source 1..23: mol_type = other DNA
caaagcccattccctctttagcc

SEQ ID NO: 351 - DNA, 23 bp, Homo sapiens
  source 1..23: mol_type = other DNA
gtcccaggaggatggcctggctg

SEQ ID NO: 352 - DNA, 23 bp, Homo sapiens
  source 1..23: mol_type = other DNA
aggaggatggcctggctgatgag

SEQ ID NO: 353 - DNA, 23 bp, Homo sapiens
  source 1..23: mol_type = other DNA
atctgtagcctctgggtctcctc

SEQ ID NO: 354 - DNA, 23 bp, Homo sapiens
  source 1..23: mol_type = other DNA
tggcttcttggtgaagatgagca

SEQ ID NO: 355 - DNA, 23 bp, Homo sapiens
  source 1..23: mol_type = other DNA
tcaatgtactccacatggggcaa

SEQ ID NO: 356 - DNA, 23 bp, Homo sapiens
  source 1..23: mol_type = other DNA
tgggatgctctgggcgaagacaa

SEQ ID NO: 357 - DNA, 23 bp, Homo sapiens
  source 1..23: mol_type = other DNA
gatgggcaccctggatgctggta

SEQ ID NO: 358 - DNA, 23 bp, Homo sapiens
  source 1..23: mol_type = other DNA
ggccgctgaccacacctgccagg

SEQ ID NO: 359 - DNA, 23 bp, Homo sapiens
  source 1..23: mol_type = other DNA
gatgggcacccactgctctgcgt

SEQ ID NO: 360 - DNA, 23 bp, Homo sapiens
  source 1..23: mol_type = other DNA
ttcaatctgtagcctctgggtct

SEQ ID NO: 361 - DNA, 23 bp, Homo sapiens
  source 1..23: mol_type = other DNA
tgacctcttccctggcttcttgg

SEQ ID NO: 362 - DNA, 23 bp, Homo sapiens
  source 1..23: mol_type = other DNA
tcttcgcccagagcatcccatgg

SEQ ID NO: 363 - DNA, 122 bp, synthetic construct; identical to SEQ ID NO: 107
  misc_feature 1..122: note = Synthetic oligonucleotide
  source 1..122: mol_type = other DNA

SEQ ID NO: 364 - DNA, 94 bp, synthetic construct; identical to SEQ ID NO: 108
  misc_feature 1..94: note = Synthetic Oligonucleotide
  source 1..94: mol_type = other DNA

SEQ ID NO: 365 - DNA, 9464 bp, synthetic construct
  misc_feature 1..9464: note = Synthetic Oligonucleotide
  source 1..9464: mol_type = other DNA
gacggatcgggagatctcccgatcccctatggtgcactctcagtacaatctgctctgatgccgcatagttaagccagtatctgctccctgcttgtgtgttggaggtcgctgagtagtgcgcgagcaaaatttaagctacaacaaggcaaggcttgaccgacaattgcatgaagaatctgcttagggttaggcgttttgcgctgcttcgcgatgtacgggccagatatacgcgttgacattgattattgactagttattaatagtaatcaattacggggtcattagttcatagcccatatatggagttccgcgttacataacttacggtaaatggcccgcctggctgaccgcccaacgacccccgcccattgacgtcaataatgacgtatgttcccatagtaacgccaatagggactttccattgacgtcaatgggtggagtatttacggtaaactgcccacttggcagtacatcaagtgtatcatatgccaagtacgccccctattgacgtcaatgacggtaaatggcccgcctggcattatgcccagtacatgaccttatgggactttcctacttggcagtacatctacgtattagtcatcgctattaccatggtgatgcggttttggcagtacatcaatgggcgtggatagcggtttgactcacggggatttccaagtctccaccccattgacgtcaatgggagtttgttttggcaccaaaatcaacgggactttccaaaatgtcgtaacaactccgccccattgacgcaaatgggcggtaggcgtgtacggtgggaggtctatataagcagagctctctggctaactagagaacccactgcttactggcttatcgaaattaatacgactcactatagggagacccaagctggctagcgtttaaacttaagcttggtaccgccaccatgacacagttcgagggctttaccaacctgtatcaggtgagcaagacactgcggtttgagctgatcccacagggcaagaccctgaagcacatccaggagcagggcttcatcgaggaggacaaggcccgcaatgatcactacaaggagctgaagcccatcatcgatcggatctacaagacctatgccgaccagtgcctgcagctggtgcagctggattgggagaacctgagcgccgccatcgactcctatagaaaggagaaaaccgaggagacaaggaacgccctgatcgaggagcaggccacatatcgcaatgccatccacgactacttcatcggccggacagacaacctgaccgatgccatcaataagagacacgccgagatctacaagggcctgttcaaggccgagctgtttaatggcaaggtgctgaagcagctgggcaccgtgaccacaaccgagcacgagaacgccctgctgcggagcttcgacaagtttacaacctacttctccggcttttatgagaacaggaagaacgtgttcagcgccgaggatatcagcacagccatcccacaccgcatcgtgcaggacaacttccccaagtttaaggagaattgtcacatcttcacacgcctgatcaccgccgtgcccagcctgcgggagcactttgagaacgtgaagaaggccatcggcatcttcgtgagcacctccatcgaggaggtgttttccttccctttttataaccagctgctgacacagacccagatcgacctgtataaccagctgctgggaggaatctctcgggaggcaggcaccgagaagatcaagggcctgaacgaggtgctgaatctggccatccagaagaatgatgagacagcccacatcatcgcctccctgccacacagattcatccccctgtttaagcagatcctgtccgataggaacaccctgtctttcatcctggaggagtttaagagcgacgaggaagtgatccagtccttctgcaagtacaagacactgctgagaaacgagaacgtgctggagacagccgaggccctgtttaacgagctgaacagcatcgacctgacacacatcttcatcagccacaagaagctggagacaatcagcagcgccctgtgcgaccactgggatacactgaggaatgccctgtatgagcggagaatctccgagctgacaggcaagatcaccaagtctgccaaggagaaggtgcagcgcagcctgaagcacgaggatatcaacctgcaggagatcatctctgccgcaggcaaggagctgagcgaggccttcaagcagaaaaccagcgagatcctgtcccacgcacacgccgccctggatcagccactgcctacaaccctgaagaagcaggaggagaaggagatcctgaagtctcagctggacagcctgctgggcctgtaccacctgctggactggtttgccgtggatgagtccaacgaggtggaccccgagttctctgcccggctgaccggcatcaagctggagatggagccgtctctgagcttctacaacaaggccagaaattatgccaccaagaagccctactccgtggagaagttcaagctgaactttcagatgcctacactggcccggggctgggacgtgaataaggagaagaacaatggcgccatcctgtttgtgaagaacggcctgtactatctgggcatcatgccaaagcagaagggcaggtataaggccctcagcttcgagcccacagagaaaaccagcgagggctttgataagatgtactatgactactttccggatgccgccaagatgatcccacggtgcagcacccagctgaaggcggtgaccgcccactttcagacccacacaacccccatcctgctgtccaacaatttcatcgagcctctggagatcacaaaggagatctacgacctgaacaatcctgagaaggagccaaagaagtttcagacagcgtacgccaagaaaaccggcgaccagaagggctacagagaggccctgtgcaagtggatcgacttcacaagggattttctgtccaagtataccaagacaacctctatcgatctgtctagcctgcggccatcctctcagtataaggacctgggcgagtactatgccgagctgaatcccctgctgtaccacatcagcttccagagaatcgccgagaaggagatcatggatgccgtggagacaggcaagctgtacctgttccagatctataacaaggactttgccaagggccaccacggcaagcctaatctgcacacactgtattggaccggtctgttttctccagagaacctggccaagacaagcatcaagctgaatggccaggccgagctgttctaccgccctaagtccaggatgaagaggatggcacaccggctgggagagaagatgctgaacaagaagctgaaggatcagaaaaccccaatccccgacaccctgtaccaggagctgtacgactatgtgaatcacagactgtcccacgacctgtctgatgaggccagggccctgctgcccaacgtgatcaccaaggaggtgtctcacgagatcatcaaggataggcgctttaccagcgacaagttctttttccacgtgcctatcacactgaactatcaggccgccaattccccatctaagttcaaccagagggtgaatgcctacctgaaggagcaccccgagacacctatcatcggcatcgatcggggcgagagaaacctgatctatatcacagtgatcgactccaccggcaagatcctggagcagcggagcctgaacaccatccagcagtttgattaccagaagaagctggacaacagggagaaggagagggtggcagcaaggcaggcctggtctgtggtgggcacaatcaaggatctgaagcagggctatctgagccaggtcatccacgagatcgtggacctgatgatccactaccaggccgtggtggtgctggagaacctgaatttcggctttaagagcaagaggaccggcatcgccgagaaggccgtgtaccagcagttcgagaagatgctgatcgataagctgaattgcctggtgctgaaggactatccagcagagaaagtgggaggcgtgctgaacccataccagctgacagaccagttcacctcctttgccaagatgggcacccagtctggcttcctgttttacgtgcctgccccatatacatctaagatcgatcccctgaccggcttcgtggaccccttcgtgtggaaaaccatcaagaatcacgagagccgcaagcacttcctggagggcttcgactttctgcactacgacgtgaaaaccggcgacttcatcctgcactttaagatgaacagaaatctgtccttccagaggggcctgcccggctttatgcctgcatgggatatcgtgttcgagaagaacgagacacagtttgacgccaagggcacccctttcatcgccggcaagagaatcgtgccagtgatcgagaatcacagattcaccggcagataccgggacctgtatcctgccaacgagctgatcgccctgctggaggagaagggcatcgtgttcagggatggctccaacatcctgccaaagctgctggagaatgacgattctcacgccatcgacaccatggtggccctgatccgcagcgtgctgcagatgcggaactccaatgccgccacaggcgaggactatatcaacagccccgtgcgcgatctgaatggcgtgtgcttcgactcccggtttcagaacccagagtggcccatggacgccgatgccaatggcgcctaccacatcgccctgaagggccagctgctgctgaatcacctgaaggagagcaaggatctgaagctgcagaacggcatctccaatcaggactggctggcctacatccaggagctgcgcaacaaaaggccggcggccacgaaaaaggccggccaggcaaaaaagaaaaagggatcctacccatacgatgttccagattacgcttatccctacgacgtgcctgattatgcatacccatatgatgtccccgactatgcctaagaattctgcagatatccagcacagtggcggccgctcgagtctagagggcccgtttaaacccgctgatcagcctcgactgtgccttctagttgccagccatctgttgtttgcccctcccccgtgccttccttgaccctggaaggtgccactcccactgtcctttcctaataaaatgaggaaattgcatcgcattgtctgagtaggtgtcattctattctggggggtggggtggggcaggacagcaagggggaggattgggaagacaatagcaggcatgctggggatgcggtgggctctatggcttctgaggcggaaagaaccagctggggctctagggggtatccccacgcgccctgtagcggcgcattaagcgcggcgggtgtggtggttacgcgcagcgtgaccgctacacttgccagcgccctagcgcccgctcctttcgctttcttcccttcctttctcgccacgttcgccggctttccccgtcaagctctaaatcgggggctccctttagggttccgatttagtgctttacggcacctcgaccccaaaaaacttgattagggtgatggttcacgtagtgggccatcgccctgatagacggtttttcgccctttgacgttggagtccacgttctttaatagtggactcttgttccaaactggaacaacactcaaccctatctcggtctattcttttgatttataagggattttgccgatttcggcctattggttaaaaaatgagctgatttaacaaaaatttaacgcgaattaattctgtggaatgtgtgtcagttagggtgtggaaagtccccaggctccccagcaggcagaagtatgcaaagcatgcatctcaattagtcagcaaccaggtgtggaaagtccccaggctccccagcaggcagaagtatgcaaagcatgcatctcaattagtcagcaaccatagtcccgcccctaactccgcccatcccgcccctaactccgcccagttccgcccattctccgccccatggctgactaattttttttatttatgcagaggccgaggccgcctctgcctctgagctattccagaagtagtgaggaggcttttttggaggcctaggcttttgcaaaaagctcccgggagcttgtatatccattttcggatctgatcaagagacaggatgaggatcgtttcgcatgattgaacaagatggattgcacgcaggttctccggccgcttgggtggagaggctattcggctatgactgggcacaacagacaatcggctgctctgatgccgccgtgttccggctgtcagcgcaggggcgcccggttctttttgtcaagaccgacctgtccggtgccctgaatgaactgcaggacgaggcagcgcggctatcgtggctggccacgacgggcgttccttgcgcagctgtgctcgacgttgtcactgaagcgggaagggactggctgctattgggcgaagtgccggggcaggatctcctgtcatctcaccttgctcctgccgagaaagtatccatcatggctgatgcaatgcggcggctgcatacgcttgatccggctacctgcccattcgaccaccaagcgaaacatcgcatcgagcgagcacgtactcggatggaagccggtcttgtcgatcaggatgatctggacgaagagcatcaggggctcgcgccagccgaactgttcgccaggctcaaggcgcgcatgcccgacggcgaggatctcgtcgtgacccatggcgatgcctgcttgccgaatatcatggtggaaaatggccgcttttctggattcatcgactgtggccggctgggtgtggcggaccgctatcaggacatagcgttggctacccgtgatattgctgaagagcttggcggcgaatgggctgaccgcttcctcgtgctttacggtatcgccgctcccgattcgcagcgcatcgccttctatcgccttcttgacgagttcttctgagcgggactctggggttcgaaatgaccgaccaagcgacgcccaacctgccatcacgagatttcgattccaccgccgccttctatgaaaggttgggcttcggaatcgttttccgggacgccggctggatgatcctccagcgcggggatctcatgctggagttcttcgcccaccccaacttgtttattgcagcttataatggttacaaataaagcaatagcatcacaaatttcacaaataaagcatttttttcactgcattctagttgtggtttgtccaaactcatcaatgtatcttatcatgtctgtataccgtcgacctctagctagagcttggcgtaatcatggtcatagctgtttcctgtgtgaaattgttatccgctcacaattccacacaacatacgagccggaagcataaagtgtaaagcctggggtgcctaatgagtgagctaactcacattaattgcgttgcgctcactgcccgctttccagtcgggaaacctgtcgtgccagctgcattaatgaatcggccaacgcgcggggagaggcggtttgcgtattgggcgctcttccgcttcctcgctcactgactcgctgcgctcggtcgttcggctgcggcgagcggtatcagctcactcaaaggcggtaatacggttatccacagaatcaggggataacgcaggaaagaacatgtgagcaaaaggccagcaaaaggccaggaaccgtaaaaaggccgcgttgctggcgtttttccataggctccgcccccctgacgagcatcacaaaaatcgacgctcaagtcagaggtggcgaaacccgacaggactataaagataccaggcgtttccccctggaagctccctcgtgcgctctcctgttccgaccctgccgcttaccggatacctgtccgcctttctcccttcgggaagcgtggcgctttctcatagctcacgctgtaggtatctcagttcggtgtaggtcgttcgctccaagctgggctgtgtgcacgaaccccccgttcagcccgaccgctgcgccttatccggtaactatcgtcttgagtccaacccggtaagacacgacttatcgccactggcagcagccactggtaacaggattagcagagcgaggtatgtaggcggtgctacagagttcttgaagtggtggcctaactacggctacactagaagaacagtatttggtatctgcgctctgctgaagccagttaccttcggaaaaagagttggtagctcttgatccggcaaacaaaccaccgctggtagcggtttttttgtttgcaagcagcagattacgcgcagaaaaaaaggatctcaagaagatcctttgatcttttctacggggtctgacgctcagtggaacgaaaactcacgttaagggattttggtcatgagattatcaaaaaggatcttcacctagatccttttaaattaaaaatgaagttttaaatcaatctaaagtatatatgagtaaacttggtctgacagttaccaatgcttaatcagtgaggcacctatctcagcgatctgtctatttcgttcatccatagttgcctgactccccgtcgtgtagataactacgatacgggagggcttaccatctggccccagtgctgcaatgataccgcgagacccacgctcaccggctccagatttatcagcaataaaccagccagccggaagggccgagcgcagaagtggtcctgcaactttatccgcctccatccagtctattaattgttgccgggaagctagagtaagtagttcgccagttaatagtttgcgcaacgttgttgccattgctacaggcatcgtggtgtcacgctcgtcgtttggtatggcttcattcagctccggttcccaacgatcaaggcgagttacatgatcccccatgttgtgcaaaaaagcggttagctccttcggtcctccgatcgttgtcagaagtaagttggccgcagtgttatcactcatggttatggcagcactgcataattctcttactgtcatgccatccgtaagatgcttttctgtgactggtgagtactcaaccaagtcattctgagaatagtgtatgcggcgaccgagttgctcttgcccggcgtcaatacgggataataccgcgccacatagcagaactttaaaagtgctcatcattggaaaacgttcttcggggcgaaaactctcaaggatcttaccgctgttgagatccagttcgatgtaacccactcgtgcacccaactgatcttcagcatcttttactttcaccagcgtttctgggtgagcaaaaacaggaaggcaaaatgccgcaaaaaagggaataagggcgacacggaaatgttgaatactcatactcttcctttttcaatattattgaagcatttatcagggttattgtctcatgagcggatacatatttgaatgtatttagaaaaataaacaaataggggttccgcgcacatttccccgaaaagtgccacctgacgtc

SEQ ID NO: 366 - DNA, 9464 bp, synthetic construct
  misc_feature 1..9464: note = Synthetic Oligonucleotide
  source 1..9464: mol_type = other DNA
gacgtcaggtggcacttttcggggaaatgtgcgcggaacccctatttgtttatttttctaaatacattcaaatatgtatccgctcatgagacaataaccctgataaatgcttcaataatattgaaaaaggaagagtatgagtattcaacatttccgtgtcgcccttattcccttttttgcggcattttgccttcctgtttttgctcacccagaaacgctggtgaaagtaaaagatgctgaagatcagttgggtgcacgagtgggttacatcgaactggatctcaacagcggtaagatccttgagagttttcgccccgaagaacgttttccaatgatgagcacttttaaagttctgctatgtggcgcggtattatcccgtattgacgccgggcaagagcaactcggtcgccgcatacactattctcagaatgacttggttgagtactcaccagtcacagaaaagcatcttacggatggcatgacagtaagagaattatgcagtgctgccataaccatgagtgataacactgcggccaacttacttctgacaacgatcggaggaccgaaggagctaaccgcttttttgcacaacatgggggatcatgtaactcgccttgatcgttgggaaccggagctgaatgaagccataccaaacgacgagcgtgacaccacgatgcctgtagcaatggcaacaacgttgcgcaaactattaactggcgaactacttactctagcttcccggcaacaattaatagactggatggaggcggataaagttgcaggaccacttctgcgctcggcccttccggctggctggtttattgctgataaatctggagccggtgagcgtgggtctcgcggtatcattgcagcactggggccagatggtaagccctcccgtatcgtagttatctacacgacggggagtcaggcaactatggatgaacgaaatagacagatcgctgagataggtgcctcactgattaagcattggtaactgtcagaccaagtttactcatatatactttagattgatttaaaacttcatttttaatttaaaaggatctaggtgaagatcctttttgataatctcatgaccaaaatcccttaacgtgagttttcgttccactgagcgtcagaccccgtagaaaagatcaaaggatcttcttgagatcctttttttctgcgcgtaatctgctgcttgcaaacaaaaaaaccgctaccagcggtggtttgtttgccggatcaagagctaccaactctttttccgaaggtaactggcttcagcagagcgcagataccaaatactgttcttctagtgtagccgtagttaggccaccacttcaagaactctgtagcaccgcctacatacctcgctctgctaatcctgttaccagtggctgctgccagtggcgataagtcgtgtcttaccgggttggactcaagacgatagttaccggataaggcgcagcggtcgggctgaacggggggttcgtgcacacagcccagcttggagcgaacgacctacaccgaactgagatacctacagcgtgagctatgagaaagcgccacgcttcccgaagggagaaaggcggacaggtatccggtaagcggcagggtcggaacaggagagcgcacgagggagcttccagggggaaacgcctggtatctttatagtcctgtcgggtttcgccacctctgacttgagcgtcgatttttgtgatgctcgtcaggggggcggagcctatggaaaaacgccagcaacgcggcctttttacggttcctggccttttgctggccttttgctcacatgttctttcctgcgttatcccctgattctgtggataaccgtattaccgcctttgagtgagctgataccgctcgccgcagccgaacgaccgagcgcagcgagtcagtgagcgaggaagcggaagagcgcccaatacgcaaaccgcctctccccgcgcgttggccgattcattaatgcagctggcacgacaggtttcccgactggaaagcgggcagtgagcgcaacgcaattaatgtgagttagctcactcattaggcaccccaggctttacactttatgcttccggctcgtatgttgtgtggaattgtgagcggataacaatttcacacaggaaacagctatgaccatgattacgccaagctctagctagaggtcgacggtatacagacatgataagatacattgatgagtttggacaaaccacaactagaatgcagtgaaaaaaatgctttatttgtgaaatttgtgatgctattgctttatttgtaaccattataagctgcaataaacaagttggggtgggcgaagaactccagcatgagatccccgcgctggaggatcatccagccggcgtcccggaaaacgattccgaagcccaacctttcatagaaggcggcggtggaatcgaaatctcgtgatggcaggttgggcgtcgcttggtcggtcatttcgaaccccagagtcccgctcagaagaactcgtcaagaaggcgatagaaggcgatgcgctgcgaatcgggagcggcgataccgtaaagcacgaggaagcggtcagcccattcgccgccaagctcttcagcaatatcacgggtagccaacgctatgtcctgatagcggtccgccacacccagccggccacagtcgatgaatccagaaaagcggccattttccaccatgatattcggcaagcaggcatcgccatgggtcacgacgagatcctcgccgtcgggcatgcgcgccttgagcctggcgaacagttcggctggcgcgagcccctgatgctcttcgtccagatcatcctgatcgacaagaccggcttccatccgagtacgtgctcgctcgatgcgatgtttcgcttggtggtcgaatgggcaggtagccggatcaagcgtatgcagccgccgcattgcatcagccatgatggatactttctcggcaggagcaaggtgagatgacaggagatcctgccccggcacttcgcccaatagcagccagtcccttcccgcttcagtgacaacgtcgagcacagctgcgcaaggaacgcccgtcgtggccagccacgatagccgcgctgcctcgtcctgcagttcattcagggcaccggacaggtcggtcttgacaaaaagaaccgggcgcccctgcgctgacagccggaacacggcggcatcagagcagccgattgtctgttgtgcccagtcatagccgaatagcctctccacccaagcggccggagaacctgcgtgcaatccatcttgttcaatcatgcgaaacgatcctcatcctgtctcttgatcagatccgaaaatggatatacaagctcccgggagctttttgcaaaagcctaggcctccaaaaaagcctcctcactacttctggaatagctcagaggcagaggcggcctcggcctctgcataaataaaaaaaattagtcagccatggggcggagaatgggcggaactgggcggagttaggggcgggatgggcggagttaggggcgggactatggttgctgactaattgagatgcatgctttgcatacttctgcctgctggggagcctggggactttccacacctggttgctgactaattgagatgcatgctttgcatacttctgcctgctggggagcctggggactttccacaccctaactgacacacattccacagaattaattcgcgttaaatttttgttaaatcagctcattttttaaccaataggccgaaatcggcaaaatcccttataaatcaaaagaatagaccgagatagggttgagtgttgttccagtttggaacaagagtccactattaaagaacgtggactccaacgtcaaagggcgaaaaaccgtctatcagggcgatggcccactacgtgaaccatcaccctaatcaagttttttggggtcgaggtgccgtaaagcactaaatcggaaccctaaagggagcccccgatttagagcttgacggggaaagccggcgaacgtggcgagaaaggaagggaagaaagcgaaaggagcgggcgctagggcgctggcaagtgtagcggtcacgctgcgcgtaaccaccacacccgccgcgcttaatgcgccgctacagggcgcgtggggataccccctagagccccagctggttctttccgcctcagaagccatagagcccaccgcatccccagcatgcctgctattgtcttcccaatcctcccccttgctgtcctgccccaccccaccccccagaatagaatgacacctactcagacaatgcgatgcaatttcctcattttattaggaaaggacagtgggagtggcaccttccagggtcaaggaaggcacgggggaggggcaaacaacagatggctggcaactagaaggcacagtcgaggctgatcagcgggtttaaacgggccctctagactcgagcggccgccactgtgctggatatctgcagaattcttaggcatagtcggggacatcatatgggtatgcataatcaggcacgtcgtagggataagcgtaatctggaacatcgtatgggtaggatccctttttcttttttgcctggccggcctttttcgtggccgccggccttttgttgcgcagctcctggatgtaggccagccagtcctgattggagatgccgttctgcagcttcagatccttgctctccttcaggtgattcagcagcagctggcccttcagggcgatgtggtaggcgccattggcatcggcgtccatgggccactctgggttctgaaaccgggagtcgaagcacacgccattcagatcgcgcacggggctgttgatatagtcctcgcctgtggcggcattggagttccgcatctgcagcacgctgcggatcagggccaccatggtgtcgatggcgtgagaatcgtcattctccagcagctttggcaggatgttggagccatccctgaacacgatgcccttctcctccagcagggcgatcagctcgttggcaggatacaggtcccggtatctgccggtgaatctgtgattctcgatcactggcacgattctcttgccggcgatgaaaggggtgcccttggcgtcaaactgtgtctcgttcttctcgaacacgatatcccatgcaggcataaagccgggcaggcccctctggaaggacagatttctgttcatcttaaagtgcaggatgaagtcgccggttttcacgtcgtagtgcagaaagtcgaagccctccaggaagtgcttgcggctctcgtgattcttgatggttttccacacgaaggggtccacgaagccggtcaggggatcgatcttagatgtatatggggcaggcacgtaaaacaggaagccagactgggtgcccatcttggcaaaggaggtgaactggtctgtcagctggtatgggttcagcacgcctcccactttctctgctggatagtccttcagcaccaggcaattcagcttatcgatcagcatcttctcgaactgctggtacacggccttctcggcgatgccggtcctcttgctcttaaagccgaaattcaggttctccagcaccaccacggcctggtagtggatcatcaggtccacgatctcgtggatgacctggctcagatagccctgcttcagatccttgattgtgcccaccacagaccaggcctgccttgctgccaccctctccttctccctgttgtccagcttcttctggtaatcaaactgctggatggtgttcaggctccgctgctccaggatcttgccggtggagtcgatcactgtgatatagatcaggtttctctcgccccgatcgatgccgatgataggtgtctcggggtgctccttcaggtaggcattcaccctctggttgaacttagatggggaattggcggcctgatagttcagtgtgataggcacgtggaaaaagaacttgtcgctggtaaagcgcctatccttgatgatctcgtgagacacctccttggtgatcacgttgggcagcagggccctggcctcatcagacaggtcgtgggacagtctgtgattcacatagtcgtacagctcctggtacagggtgtcggggattggggttttctgatccttcagcttcttgttcagcatcttctctcccagccggtgtgccatcctcttcatcctggacttagggcggtagaacagctcggcctggccattcagcttgatgcttgtcttggccaggttctctggagaaaacagaccggtccaatacagtgtgtgcagattaggcttgccgtggtggcccttggcaaagtccttgttatagatctggaacaggtacagcttgcctgtctccacggcatccatgatctccttctcggcgattctctggaagctgatgtggtacagcaggggattcagctcggcatagtactcgcccaggtccttatactgagaggatggccgcaggctagacagatcgatagaggttgtcttggtatacttggacagaaaatcccttgtgaagtcgatccacttgcacagggcctctctgtagcccttctggtcgccggttttcttggcgtacgctgtctgaaacttctttggctccttctcaggattgttcaggtcgtagatctcctttgtgatctccagaggctcgatgaaattgttggacagcaggatgggggttgtgtgggtctgaaagtgggcggtcaccgccttcagctgggtgctgcaccgtgggatcatcttggcggcatccggaaagtagtcatagtacatcttatcaaagccctcgctggttttctctgtgggctcgaagctgagggccttatacctgcccttctgctttggcatgatgcccagatagtacaggccgttcttcacaaacaggatggcgccattgttcttctccttattcacgtcccagccccgggccagtgtaggcatctgaaagttcagcttgaacttctccacggagtagggcttcttggtggcataatttctggccttgttgtagaagctcagagacggctccatctccagcttgatgccggtcagccgggcagagaactcggggtccacctcgttggactcatccacggcaaaccagtccagcaggtggtacaggcccagcaggctgtccagctgagacttcaggatctccttctcctcctgcttcttcagggttgtaggcagtggctgatccagggcggcgtgtgcgtgggacaggatctcgctggttttctgcttgaaggcctcgctcagctccttgcctgcggcagagatgatctcctgcaggttgatatcctcgtgcttcaggctgcgctgcaccttctccttggcagacttggtgatcttgcctgtcagctcggagattctccgctcatacagggcattcctcagtgtatcccagtggtcgcacagggcgctgctgattgtctccagcttcttgtggctgatgaagatgtgtgtcaggtcgatgctgttcagctcgttaaacagggcctcggctgtctccagcacgttctcgtttctcagcagtgtcttgtacttgcagaaggactggatcacttcctcgtcgctcttaaactcctccaggatgaaagacagggtgttcctatcggacaggatctgcttaaacagggggatgaatctgtgtggcagggaggcgatgatgtgggctgtctcatcattcttctggatggccagattcagcacctcgttcaggcccttgatcttctcggtgcctgcctcccgagagattcctcccagcagctggttatacaggtcgatctgggtctgtgtcagcagctggttataaaaagggaaggaaaacacctcctcgatggaggtgctcacgaagatgccgatggccttcttcacgttctcaaagtgctcccgcaggctgggcacggcggtgatcaggcgtgtgaagatgtgacaattctccttaaacttggggaagttgtcctgcacgatgcggtgtgggatggctgtgctgatatcctcggcgctgaacacgttcttcctgttctcataaaagccggagaagtaggttgtaaacttgtcgaagctccgcagcagggcgttctcgtgctcggttgtggtcacggtgcccagctgcttcagcaccttgccattaaacagctcggccttgaacaggcccttgtagatctcggcgtgtctcttattgatggcatcggtcaggttgtctgtccggccgatgaagtagtcgtggatggcattgcgatatgtggcctgctcctcgatcagggcgttccttgtctcctcggttttctcctttctataggagtcgatggcggcgctcaggttctcccaatccagctgcaccagctgcaggcactggtcggcataggtcttgtagatccgatcgatgatgggcttcagctccttgtagtgatcattgcgggccttgtcctcctcgatgaagccctgctcctggatgtgcttcagggtcttgccctgtgggatcagctcaaaccgcagtgtcttgctcacctgatacaggttggtaaagccctcgaactgtgtcatggtggcggtaccaagcttaagtttaaacgctagccagcttgggtctccctatagtgagtcgtattaatttcgataagccagtaagcagtgggttctctagttagccagagagctctgcttatatagacctcccaccgtacacgcctaccgcccatttgcgtcaatggggcggagttgttacgacattttggaaagtcccgttgattttggtgccaaaacaaactcccattgacgtcaatggggtggagacttggaaatccccgtgagtcaaaccgctatccacgcccattgatgtactgccaaaaccgcatcaccatggtaatagcgatgactaatacgtagatgtactgccaagtaggaaagtcccataaggtcatgtactgggcataatgccaggcgggccatttaccgtcattgacgtcaatagggggcgtacttggcatatgatacacttgatgtactgccaagtgggcagtttaccgtaaatactccacccattgacgtcaatggaaagtccctattggcgttactatgggaacatacgtcattattgacgtcaatgggcgggggtcgttgggcggtcagccaggcgggccatttaccgtaagttatgtaacgcggaactccatatatgggctatgaactaatgaccccgtaattgattactattaataactagtcaataatcaatgtcaacgcgtatatctggcccgtacatcgcgaagcagcgcaaaacgcctaaccctaagcagattcttcatgcaattgtcggtcaagccttgccttgttgtagcttaaattttgctcgcgcactactcagcgacctccaacacacaagcagggagcagatactggcttaactatgcggcatcagagcagattgtactgagagtgcaccataggggatcgggagatctcccgatccgtc

SEQ ID NO: 367 - protein, 1352 aa, Homo sapiens
MTQFEGFTNLYQVSKTLRFELIPQGKTLKHIQEQGFIEEDKARNDHYKELKPIIDRIYKTYADQCLQLVQLDWENLSAAIDSYRKEKTEETRNALIEEQATYRNAIHDYFIGRTDNLTDAINKRHAEIYKGLFKAELFNGKVLKQLGTVTTTEHENALLRSFDKFTTYFSGFYENRKNVFSAEDISTAIPHRIVQDNFPKFKENCHIFTRLITAVPSLREHFENVKKAIGIFVSTSIEEVFSFPFYNQLLTQTQIDLYNQLLGGISREAGTEKIKGLNEVLNLAIQKNDETAHIIASLPHRFIPLFKQILSDRNTLSFILEEFKSDEEVIQSFCKYKTLLRNENVLETAEALFNELNSIDLTHIFISHKKLETISSALCDHWDTLRNALYERRISELTGKITKSAKEKVQRSLKHEDINLQEIISAAGKELSEAFKQKTSEILSHAHAALDQPLPTTLKKQEEKEILKSQLDSLLGLYHLLDWFAVDESNEVDPEFSARLTGIKLEMEPSLSFYNKARNYATKKPYSVEKFKLNFQMPTLARGWDVNKEKNNGAILFVKNGLYYLGIMPKQKGRYKALSFEPTEKTSEGFDKMYYDYFPDAAKMIPRCSTQLKAVTAHFQTHTTPILLSNNFIEPLEITKEIYDLNNPEKEPKKFQTAYAKKTGDQKGYREALCKWIDFTRDFLSKYTKTTSIDLSSLRPSSQYKDLGEYYAELNPLLYHISFQRIAEKEIMDAVETGKLYLFQIYNKDFAKGHHGKPNLHTLYWTGLFSPENLAKTSIKLNGQAELFYRPKSRMKRMAHRLGEKMLNKKLKDQKTPIPDTLYQELYDYVNHRLSHDLSDEARALLPNVITKEVSHEIIKDRRFTSDKFFFHVPITLNYQAANSPSKFNQRVNAYLKEHPETPIIGIDRGERNLIYITVIDSTGKILEQRSLNTIQQFDYQKKLDNREKERVAARQAWSVVGTIKDLKQGYLSQVIHEIVDLMIHYQAVVVLENLNFGFKSKRTGIAEKAVYQQFEKMLIDKLNCLVLKDYPAEKVGGVLNPYQLTDQFTSFAKMGTQSGFLFYVPAPYTSKIDPLTGFVDPFVWKTIKNHESRKHFLEGFDFLHYDVKTGDFILHFKMNRNLSFQRGLPGFMPAWDIVFEKNETQFDAKGTPFIAGKRIVPVIENHRFTGRYRDLYPANELIALLEEKGIVFRDGSNILPKLLENDDSHAIDTMVALIRSVLQMRNSNAATGEDYINSPVRDLNGVCFDSRFQNPEWPMDADANGAYHIALKGQLLLNHLKESKDLKLQNGISNQDWLAYIQELRNKRPAATKKAGQAKKKKGSYPYDVPDYAYPYDVPDYAYPYDVPDYA

SEQ ID NO: 368 - protein, 5 aa, synthetic construct
APRPG

SEQ ID NO: 369 - protein, 5 aa, synthetic construct
ASSHN

SEQ ID NO: 370 - protein, 6 aa, synthetic construct
KCCYSL

SEQ ID NO: 371 - protein, 7 aa, synthetic construct
YEVGHRC

SEQ ID NO: 372 - protein, 12 aa, synthetic construct
GGGSGGGSGGGS

SEQ ID NO: 373 - protein, 7 aa, synthetic construct
AEAAAKA